European Patent Specification EP 3 193 905 B1, published April 3, 2024. Title: Methods of Treating Cervical Cancer. Applicant: GENEXINE, INC. Hyun-Tak, JIN Hye Seong, LIM You Suk, SUH Eun Joo, NAM. The sequence listing filed with the application follows.

SEQUENCE LISTING (116 sequences)

SEQ ID NO: 1 - DNA, 477 bp, Human papillomavirus 16
  misc_feature: E6 nucleotide sequence
atgcaccaaaagagaactgcaatgtttcaggacccacaggagcgacccagaaagttaccacatttatgcacagagctgcaaacaactatacatgatataatattagaatgtgtgtactgcaagcaacagttactgcgacgtgaggtatatgactttgcttttcgggatttatgcatagtatatagagatgggaatccatatgcagtgtgtgataaatgtttaaagttttattctaaaattagtgagtatagatattattgttatagtgtgtatggaacaacattagaacagcaatacaacaaaccgttgtgtgatttgttaattaggtgtattaactgtcaaaagccactgtgtcctgaagaaaagcaaagacatctggacaaaaagcaaagattccataatataaggggtcggtggaccggtcgatgtatgtcttgttgcagatcatcaagaacacgtagagaaacccagctgtaa

SEQ ID NO: 2 - protein, 158 aa, Human papillomavirus 16
  MISC_FEATURE: E6 protein
MHQKRTAMFQDPQERPRKLPHLCTELQTTIHDIILECVYCKQQLLRREVYDFAFRDLCIVYRDGNPYAVCDKCLKFYSKISEYRYYCYSVYGTTLEQQYNKPLCDLLIRCINCQKPLCPEEKQRHLDKKQRFHNIRGRWTGRCMSCCRSSRTRRETQL

SEQ ID NO: 3 - DNA, 477 bp, Human papillomavirus 18
  misc_feature: E6 nucleotide sequence
atggcgcgctttgaggatccaacacggcgaccctacaagctacctgatctgtgcacggaactgaacacttcactgcaagacatagaaataacctgtgtatattgcaagacagtattggaacttacagaggtatttgaatttgcattcaaagatttatttgtagtgtatagagacagtataccgcatgctgcatgccataaatgtatagatttctattctagaattagagaattaagatattattcagactctgtgtatggagacacattagaaaaactaactaacactgggttatacaatttattaataaggtgcctgcggtgccagaaaccgttgaatccagcagaaaaacttagacaccttaatgaaaaacgacgattccacaaaatagctgggcactatagaggccagtgccattcgtgctgcaaccgagcacgacaggagagactccaacgacgcagagaaacacaagtataa

SEQ ID NO: 4 - protein, 158 aa, Human papillomavirus 18
  MISC_FEATURE: E6 protein
MARFEDPTRRPYKLPDLCTELNTSLQDIEITCVYCKTVLELTEVFEFAFKDLFVVYRDSIPHAACHKCIDFYSRIRELRYYSDSVYGDTLEKLTNTGLYNLLIRCLRCQKPLNPAEKLRHLNEKRRFHKIAGHYRGQCHSCCNRARQERLQRRRETQV

SEQ ID NO: 5 - DNA, 297 bp, Human papillomavirus 16
  misc_feature: E7 nucleotide sequence
atgcatggagatacacctacattgcatgaatatatgttagatttgcaaccagagacaactgatctctactgttatgagcaattaaatgacagctcagaggaggaggatgaaatagatggtccagctggacaagcagaaccggacagagcccattacaatattgtaaccttttgttgcaagtgtgactctacgcttcggttgtgcgtacaaagcacacacgtagacattcgtactttggaagacctgttaatgggcacactaggaattgtgtgccccatctgttctcagaaaccataa

SEQ ID NO: 6 - protein, 98 aa, Human papillomavirus 16
  MISC_FEATURE: E7 protein
MHGDTPTLHEYMLDLQPETTDLYCYEQLNDSSEEEDEIDGPAGQAEPDRAHYNIVTFCCKCDSTLRLCVQSTHVDIRTLEDLLMGTLGIVCPICSQKP

SEQ ID NO: 7 - DNA, 318 bp, Human papillomavirus 18
  misc_feature: E7 nucleotide sequence
atgtatggacctaaggcaacattgcaagacattgtattgcatttagagcctcaaaatgaaattccggttgaccttctatgtcacgagcaattaagcgactcagaggaagaaaacgatgaaatagatggagttaatcatcaacatttaccagcccgacgagccgaaccacaacgtcacacaatgttgtgtatgtgttgtaagtgtgaagccagaattgagctagtagtagaaagctcagcagacgaccttcgagcattccagcagctgtttctgagcaccctgtcctttgtgtgtccgtggtgtgcatcccagcagtaa

SEQ ID NO: 8 - protein, 105 aa, Human papillomavirus 18
  MISC_FEATURE: E7 protein
MYGPKATLQDIVLHLEPQNEIPVDLLCHEQLSDSEEENDEIDGVNHQHLPARRAEPQRHTMLCMCCKCEARIELVVESSADDLRAFQQLFLSTLSFVCPWCASQQ

SEQ ID NO: 9 - DNA, 1737 bp, Artificial Sequence
  codon optimized sequence of GX-188 without FLT3L and signal peptide
atgcaccagaagagaaccgccatgttccaggaccctcaggagagacctaggaagctgcctcacctgtgtacagagctccagacaaccatccacgacatcatcctggagtgcgtgtactgtaagcagcagctgctgagaagagaggtgtacgacttcgccttcagagacctgtgcatcgtgtacagagacggcaacccttacgccgtgtgcgataagtgtctgaagttctattccaaaatctccgaatataggtacatgcacggcgacacccctaccctgcacgagtacatgctggacctccagcctgagaccacagacctgtactgctacgagcagctgaacgacagctctgaggaagaggacgagattgacggacctgctggccaggccgagcctgacagagcccactacaatatcgtgacattctgttgcaaatgcgactccacactggacaagtgcctgaagttctacagcaagatctctgagtacagatactactgctactctgtgtacggcaccacactggagcagcagtacaacaagcctctgtgcgacctcctgatccgctgcatcaactgccagaagcctctgtgccctgaggagaagcagagacacctggacaagaagcagcggttccacaacatcagaggcagatggaccggcaggtgcatgtcctgctgtagatcctccagaaccagacgggagacccagctgcactacaacatcgtgaccttctgctgcaagtgcgactctaccctgagactgtgcgtgcagtctacccacgtggacatcagaaccctggaggacctgctgatgggcaccctgggcatcgtgtgccctatctgctctcagaagcctatggccaggttcgaggaccctaccagaagaccctacaagctgcctgacctgtgcaccgagctgaacacctctctgcaagacatcgagatcacctgcgtgtactgcaagaccgtgctggagctgaccgaggtgttcgagttcgccttcaaggacctgttcgtggtgtacagagacagcatccctcacgctgcctgccacaagtgcatcgacttctattccaggatcagggagctgcgctattactccgactctgtgatgtacggccccaaggccaccctccaggacatcgtgctgcacctggagcctcagaacgagatccccgtggacctgctgtgccacgagcagctgtctgactctgaagaggagaacgacgagatcgacggcgtgaaccaccagcacctgcctgccaggagagctgaaccccagcggcataccatgctgtgtatgtgcttctactctaggatcagagagctgaggtactactctgactctgtgtacggcgacaccctggagaagctgaccaacaccggcctgtacaacctgctgatccggtgcctgaggtgccagaagcctctgaaccctgccgagaagctgagacacctgaacgagaagagaagattccacaagatcgctggccactacagaggccagtgccactcttgctgcaacagagccagacaggagagactccagcggagaagggagacccaggtggccagaagagccgagcctcagagacacaccatgctgtgcatgtgctgcaagtgcgaggccagaatcgagctggtggtggagagctctgccgacgacctgagagccttccagcagctgttcctgtctaccctgagcttcgtgtgcccttggtgcgcctctcagcag

SEQ ID NO: 10 - protein, 579 aa, Artificial Sequence
  amino acid sequence of GX-188 without FLT3L and signal peptide
MHQKRTAMFQDPQERPRKLPHLCTELQTTIHDIILECVYCKQQLLRREVYDFAFRDLCIVYRDGNPYAVCDKCLKFYSKISEYRYMHGDTPTLHEYMLDLQPETTDLYCYEQLNDSSEEEDEIDGPAGQAEPDRAHYNIVTFCCKCDSTLDKCLKFYSKISEYRYYCYSVYGTTLEQQYNKPLCDLLIRCINCQKPLCPEEKQRHLDKKQRFHNIRGRWTGRCMSCCRSSRTRRETQLHYNIVTFCCKCDSTLRLCVQSTHVDIRTLEDLLMGTLGIVCPICSQKPMARFEDPTRRPYKLPDLCTELNTSLQDIEITCVYCKTVLELTEVFEFAFKDLFVVYRDSIPHAACHKCIDFYSRIRELRYYSDSVMYGPKATLQDIVLHLEPQNEIPVDLLCHEQLSDSEEENDEIDGVNHQHLPARRAEPQRHTMLCMCFYSRIRELRYYSDSVYGDTLEKLTNTGLYNLLIRCLRCQKPLNPAEKLRHLNEKRRFHKIAGHYRGQCHSCCNRARQERLQRRRETQVARRAEPQRHTMLCMCCKCEARIELVVESSADDLRAFQQLFLSTLSFVCPWCASQQ

SEQ ID NO: 11 - DNA, 489 bp, Artificial Sequence
  Nucleotide sequence of FLT3L  (fms-like tyrosine kinase-3 ligand)
atcacccaggactgctccttccaacacagccccatctcctccgacttcgctgtcaaaatccgtgagctgtctgactacctgcttcaagattacccagtcaccgtggcctccaacctgcaggacgaggagctctgcgggggcctctggcggctggtcctggcacagcgctggatggagcggctcaagactgtcgctgggtccaagatgcaaggcttgctggagcgcgtgaacacggagatacactttgtcaccaaatgtgcctttcagcccccccccagctgtcttcgcttcgtccagaccaacatctcccgcctcctgcaggagacctccgagcagctggtggcgctgaagccctggatcactcgccagaacttctcccggtgcctggagctgcagtgtcagcccgactcctcaaccctgccacccccatggagtccccggcccctggaggccacagccccgacagccccgggcggcggcagcggcgat

SEQ ID NO: 12 - protein, 163 aa, Artificial Sequence
  Amino acid sequence of FLT3L  (fms-like tyrosine kinase-3 ligand)
ITQDCSFQHSPISSDFAVKIRELSDYLLQDYPVTVASNLQDEELCGGLWRLVLAQRWMERLKTVAGSKMQGLLERVNTEIHFVTKCAFQPPPSCLRFVQTNISRLLQETSEQLVALKPWITRQNFSRCLELQCQPDSSTLPPPWSPRPLEATAPTAPGGGSGD

SEQ ID NO: 13 - DNA, 69 bp, Artificial Sequence
  Signal peptide of tPA
atggatgctatgaaacggggcctgtgctgcgtgctgctcctgtgcggcgctgtgtttgtgagccctagc

SEQ ID NO: 14 - protein, 23 aa, Artificial Sequence
  Signal peptide of tPA
MDAMKRGLCCVLLLCGAVFVSPS

SEQ ID NO: 15 - DNA, 6085 bp, Artificial Sequence
  GX-188E
acgcgttgacattgattattgactagttattaatagtaatcaattacggggtcattagttcatagcccatatatggagttccgcgttacataacttacggtaaatggcccgcctggctgaccgcccaacgacccccgcccattgacgtcaataatgacgtatgttcccatagtaacgccaatagggactttccattgacgtcaatgggtggagtatttacggtaaactgcccacttggcagtacatcaagtgtatcatatgccaagtacgccccctattgacgtcaatgacggtaaatggcccgcctggcattatgcccagtacatgaccttatgggactttcctacttggcagtacatctacgtattagtcatcgctattaccatggtgatgcggttttggcagtacatcaatgggcgtggatagcggtttgactcacggggatttccaagtctccaccccattgacgtcaatgggagtttgttttggcaccaaaatcaacgggactttccaaaatgtcgtaacaactccgccccattgacgcaaatgggcggtaggcgtgtacggtgggaggtctatataagcagagctctctggctaactagagaacccactgcttactggcttatcgaaattaatacgactcactatagggagacccaagctggctagcgtgagtttggggacccttgattgttctttctttttcgctattgtaaaattcatgttatatggagggggcaaagttttcagggtgttgtttagaacgggaagatgtcccttgtatcaccatggaccctcatgataattttgtttctttcactttctactctgttgacaaccattgtctcctcttattttcttttcattttctgtaactttttcgttaaactttagcttgcatttgtaacgaatttttaaattcacttttgtttatttgtcagattgtaagtactttctctaatcacttttttttcaaggcaatcagggtatattatattgtacttcagcacagttttagagaacaattgttataattaaatgataaggtagaatatttctgcatataaattctggctggcgtggaaatattcttattggtagaaacaactacatcctggtcatcatcctgcctttctctttatggttacaatgatatacactgtttgagatgaggataaaatactctgagtccaaaccgggcccctctgctaaccatgttcatgccttcttctttttcctacagctcctgggcaacgtgctggttattgtgctgtctcatcattttggcaaagaattgtaatacgactcactatagggcgaattgaagcttggtaccgccaccatggatgctatgaaacggggcctgtgctgcgtgctgctcctgtgcggcgctgtgtttgtgagccctagcatcacccaggactgctccttccaacacagccccatctcctccgacttcgctgtcaaaatccgtgagctgtctgactacctgcttcaagattacccagtcaccgtggcctccaacctgcaggacgaggagctctgcgggggcctctggcggctggtcctggcacagcgctggatggagcggctcaagactgtcgctgggtccaagatgcaaggcttgctggagcgcgtgaacacggagatacactttgtcaccaaatgtgcctttcagcccccccccagctgtcttcgcttcgtccagaccaacatctcccgcctcctgcaggagacctccgagcagctggtggcgctgaagccctggatcactcgccagaacttctcccggtgcctggagctgcagtgtcagcccgactcctcaaccctgccacccccatggagtccccggcccctggaggccacagccccgacagccccgggcggcggcagcggcgatgctagcatgcaccagaagagaaccgccatgttccaggaccctcaggagagacctaggaagctgcctcacctgtgtacagagctccagacaaccatccacgacatcatcctggagtgcgtgtactgtaagcagcagctgctgagaagagaggtgtacgacttcgccttcagagacctgtgcatcgtgtacagagacggcaacccttacgccgtgtgcgataagtgtctgaagttctattccaaaatctccgaatataggtacatgcacggcgacacccctaccctgcacgagtacatgctggacctccagcctgagaccacagacctgtactgctacgagcagctgaacgacagctctgaggaagaggacgagattgacggacctgctggccaggccgagcctgacagagcccactacaatatcgtgacattctgttgcaaatgcgactccacactggacaagtgcctgaagttctacagcaagatctctgagtacagatactactgctactctgtgtacggcaccacactggagcagcagtacaacaagcctctgtgcgacctcctgatccgctgcatcaactgccagaagcctctgtgccctgaggagaagcagagacacctggacaagaagcagcggttccacaacatcagaggcagatggaccggcaggtgcatgtcctgctgtagatcctccagaaccagacgggagacccagctgcactacaacatcgtgaccttctgctgcaagtgcgactctaccctgagactgtgcgtgcagtctacccacgtggacatcagaaccctggaggacctgctgatgggcaccctgggcatcgtgtgccctatctgctctcagaagcctatggccaggttcgaggaccctaccagaagaccctacaagctgcctgacctgtgcaccgagctgaacacctctctgcaagacatcgagatcacctgcgtgtactgcaagaccgtgctggagctgaccgaggtgttcgagttcgccttcaaggacctgttcgtggtgtacagagacagcatccctcacgctgcctgccacaagtgcatcgacttctattccaggatcagggagctgcgctattactccgactctgtgatgtacggccccaaggccaccctccaggacatcgtgctgcacctggagcctcagaacgagatccccgtggacctgctgtgccacgagcagctgtctgactctgaagaggagaacgacgagatcgacggcgtgaaccaccagcacctgcctgccaggagagctgaaccccagcggcataccatgctgtgtatgtgcttctactctaggatcagagagctgaggtactactctgactctgtgtacggcgacaccctggagaagctgaccaacaccggcctgtacaacctgctgatccggtgcctgaggtgccagaagcctctgaaccctgccgagaagctgagacacctgaacgagaagagaagattccacaagatcgctggccactacagaggccagtgccactcttgctgcaacagagccagacaggagagactccagcggagaagggagacccaggtggccagaagagccgagcctcagagacacaccatgctgtgcatgtgctgcaagtgcgaggccagaatcgagctggtggtggagagctctgccgacgacctgagagccttccagcagctgttcctgtctaccctgagcttcgtgtgcccttggtgcgcctctcagcagtaatctagagtcggggcggccggccgcttcgagcagacatgataagatacattgatgagtttggacaaaccacaactagaatgcagtgaaaaaaatgctttatttgtgaaatttgtgatgctattgctttatttgtaaccattataagctgcaataaacaagttaacaacaacaattgcattcattttatgtttcaggttcagggggaggtgtgggaggttttttaaagcaagtaaaacctctacaaatgtggtaaaatcgataaggatctgaacgatggagcggagaatgggcggaactgggcggagttaggggcgggatgggcggagttaggggcgggactatggttgctgactaattgagatgcatgctttgcatacttctgcctgctggggagcctggggactttccacacctggttgctgactaattgagatgcatgctttgcatacttctgcctgctggggagcctggggactttccacaccctaactgacacacattccacagcggatccgtcgacttcagaagaactcgtcaagaaggcgatagaaggcgatgcgccgcgaatcgggagcggcgataccgtagagcacgaggaagcggtcagcccattcgccgccaagctcttcagcaatatcacgggtagccaacgctatgtcctgatagcggtccgccacacccagccggccacagtcgatgaatccagaaaagcggccattttccaccatgatattcggcaagcaggcatcgccatgggtcacgacgagatcctcgccgtcgggcatgctcgccttgagcctggcgaacagttcggctggcgcgagcccctgatgctcttcgtccagatcatcctgatcgacaagaccggcttccatccgagtacgtgctcgctcgatgcgatgtttcgcttggtggtcgaatgggcaggtagccggatcaagcgtatgcagccgccgcattgcatcagccatgatggatactttctcggcaggagcaaggtgagatgacaggagatcctgccccggcacttcgcccaatagcagccagtcccttcccgcttcagtgacaacgtcgagcacagctgcgcaaggaacgcccgtcgtggccagccacgatagccgcgctgcctcgtcttgcagttcattcagggcaccggacaggtcggtcttgacaaaaagaaccgggcgcccctgcgctgacagccggaacacggcggcatcagagcagccgattgtctgttgtgcccagtcatagccgaatagcctctccacccaagcggccggagaacctgcgtgcaatccatcttgttcaatcatgcgaaacgatcctcatcctgtctcttgatcagatcttgatcccctgcgccatcagatccttggcggcaagaaagccatccagtttactttgcagggcttcccaaccttaccagagggcgccccagctggcaattccggttcgcttgctgtccataaaaccgcccagtctagctatcgccatgtaagcccactgcaagctacctgctttctctttgcgcttgcgttttcccttgtccagatagcccagtagctgacattcatccggggtcagcaccgtttctgcggactggctttctacgtgaaaaggatctaggtgaagatcctttttgataatctcatgaccaaaatcccttaacgtgagttttcgttccactgagcgtcagaccccgtagaaaagatcaaaggatcttcttgagatcctttttttctgcgcgtaatctgctgcttgcaaacaaaaaaaccaccgctaccagcggtggtttgtttgccggatcaagagctaccaactctttttccgaaggtaactggcttcagcagagcgcagataccaaatactgttcttctagtgtagccgtagttaggccaccacttcaagaactctgtagcaccgcctacatacctcgctctgctaatcctgttaccagtggctgctgccagtggcgataagtcgtgtcttaccgggttggactcaagacgatagttaccggataaggcgcagcggtcgggctgaacggggggttcgtgcacacagcccagcttggagcgaacgacctacaccgaactgagatacctacagcgtgagctatgagaaagcgccacgcttcccgaagggagaaaggcggacaggtatccggtaagcggcagggtcggaacaggagagcgcacgagggagcttccagggggaaacgcccggtatctttatagtcctgtcgggtttcgccacctctgacttgagcgtcgatttttgtgatgctcgtcaggggggcggagcctatggaaaaacgccagcaacgcggcctttttacggttcctggccttttgctggccttttgctcacatgttcgggcccaatcgacccgggcgacggccagtgaattgtaccgatgtacgggccagatat

SEQ ID NO: 16 - protein, 12 aa, Artificial Sequence
  alpha-1 helix of E7 protein of HPV16 (position 73-84)
HVDIRTLEDLLM

SEQ ID NO: 17 - protein, 8 aa, Artificial Sequence
  beta-2 sheet of E7 protein of HPV16 (position 64-71)
TLRLCVQS

SEQ ID NO: 18 - protein, 11 aa, Artificial Sequence
  beta-1 sheet of E7 protein of HPV16 (position 48-58)
DRAHYNIVTFC

SEQ ID NO: 19 - protein, 151 aa, Human papillomavirus 16
  MISC_FEATURE: AAA91670.1 E6 Variant
MFQDPQERPRKLPQLCTELQTTIHDIILECVYCKQQLLRREVYDFAFRDLCIVYRDGNPYAVCDKCLKFYSKISEYRHYCYSLYGTTLEQQYNKPLCDLLIRCINCQKPLCPEEKQRHLDKKQRFHNIRGRWTGRCMSCCRSSRTRRETQL

SEQ ID NO: 20 - protein, 151 aa, Human papillomavirus 16; identical to SEQ ID NO: 19
  MISC_FEATURE: AAA91673.1 E6 Variant

SEQ ID NO: 21 - protein, 151 aa, Human papillomavirus 16
  MISC_FEATURE: AAA91669.1 E6 Variant
MFQDPQERPRKLPQLCTELQTTIHDIILECVYCKQQLLRREVYDFAFRDLCIVYKNGNPYAVCDKCLKFYSKISEYRHYCYSVYGTTLEQQYNKPLCDLLIRCINCQKPLCPEEKQRHLDKKQRFHNIRGRWTGRCMSCCRSSRTRRETQL

SEQ ID NO: 22 - protein, 151 aa, Human papillomavirus 16
  MISC_FEATURE: AAA91674.1 E6 Variant
MFQDPQERPRKLPQLCTELQTTIHDIILECVYCKQQLLRREVYDFAFRDLCIVYRDGNPYAVCDKCLKFYSKISEYRHYCYSVYGTTLEQQYNKPLCDLLIRCINCQKPLCPEEKQRHLDKKQRFHNIRGRWTGRCMSCCRSSRTRRETQL

SEQ ID NO: 23 - protein, 151 aa, Human papillomavirus 16; identical to SEQ ID NO: 22
  MISC_FEATURE: AAA91680.1 E6 Variant

SEQ ID NO: 24 - protein, 151 aa, Human papillomavirus 16; identical to SEQ ID NO: 22
  MISC_FEATURE: AAA91681.1

SEQ ID NO: 25 - protein, 151 aa, Human papillomavirus 16; identical to SEQ ID NO: 19
  MISC_FEATURE: AAA91668.1 E6 Variant

SEQ ID NO: 26 - protein, 151 aa, Human papillomavirus 16; identical to SEQ ID NO: 19
  MISC_FEATURE: AAA91658.1 E6 Variant

SEQ ID NO: 27 - protein, 151 aa, Human papillomavirus 16
  MISC_FEATURE: AAA91662.1 E6 Variant
MFQDPQERPRKLPQLCTELQTTIHEIILECVYCKQQLLRREVYDFAFRDLCIVYRDGNPYAVCDKCLKFYSKISEYRHYCYSLYGTTLEQQYNKPLCDLLIRCINCQKPLCPEEKQRHLDKKQRFHNIRGRWTGRCMSCCRSSRTRRETQL

SEQ ID NO: 28 - protein, 151 aa, Human papillomavirus 16; identical to SEQ ID NO: 27
  MISC_FEATURE: AAA91667.1 E6 Variant

SEQ ID NO: 29 - protein, 151 aa, Human papillomavirus 16; identical to SEQ ID NO: 27
  MISC_FEATURE: AAA91676.1 E6 Variant

SEQ ID NO: 30 - protein, 151 aa, Human papillomavirus 16; identical to SEQ ID NO: 27
  MISC_FEATURE: AAA91671.1 E6 Variant

SEQ ID NO: 31 - protein, 151 aa, Human papillomavirus 16
  MISC_FEATURE: AAA91656.1 E6 Variant
MFQDPQERPGKLPQLCTELQTTIHDIILECVYCKQQLLRREVYDFAFRDLCIVYRDGNPYAVCDKCLKFYSKISEYRHYCYSVYGTTLEQQYNKPLCDLLIRCINCQKPLCPEEKQRHLDKKQRFHNIRGRWTGRCMSCCRSSRTRRETQL

SEQ ID NO: 32 - protein, 151 aa, Human papillomavirus 16; identical to SEQ ID NO: 31
  MISC_FEATURE: AAA91682.1 E6 Variant

SEQ ID NO: 33 - protein, 151 aa, Human papillomavirus 16; identical to SEQ ID NO: 31
  MISC_FEATURE: AAA91657.1 E6 Variant

SEQ ID NO: 34 - protein, 151 aa, Human papillomavirus 16; identical to SEQ ID NO: 31
  MISC_FEATURE: AAA91660.1 E6 Variant

SEQ ID NO: 35 - protein, 151 aa, Human papillomavirus 16
  MISC_FEATURE: AAA91677.1 E6 Variant
MFQDPQERPTKLPDLCTELQTTIHDIILECVYCKQQLLRREVYDFAFRDLCIVYRDGNPYAVCDKCLKFYSKISEYRYYCYSLYGTTLEQQYNKPLCDLLIRCINCQKPLCPEEKQRHLDKKQRFHNIRGRWTGRCMSCCRSSRTRRETQL

SEQ ID NO: 36 - protein, 151 aa, Human papillomavirus 16; identical to SEQ ID NO: 35
  MISC_FEATURE: AAA91678.1 E6 Variant

SEQ ID NO: 37 - protein, 151 aa, Human papillomavirus 16; identical to SEQ ID NO: 35
  MISC_FEATURE: AAA91672.1 E6 Variant

SEQ ID NO: 38 - protein, 151 aa, Human papillomavirus 16; identical to SEQ ID NO: 35
  MISC_FEATURE: AAA91661.1 E6 Variant

SEQ ID NO: 39 - protein, 151 aa, Human papillomavirus 16
  MISC_FEATURE: AAA91664.1 E6 Variant
MFQDPQERPIKLPDLCTELQTTIHDIILECVYCKQQLLRREVYDFAFRDLCIVYRDGNPYAVCDKCLKFYSKISEYRYYCYSLYGTTLEQQYNKPLCDLLIRCINCQKPLCPEEKQRHLDKKQRFHNIRGRWTGRCMSCCRSSRTRRETQL

SEQ ID NO: 40 - protein, 151 aa, Human papillomavirus 16; identical to SEQ ID NO: 39
  MISC_FEATURE: AAA91675.1 E6 Variant

SEQ ID NO: 41 - protein, 151 aa, Human papillomavirus 16; identical to SEQ ID NO: 39
  MISC_FEATURE: AAA91665.1 E6 Variant

SEQ ID NO: 42 - protein, 151 aa, Human papillomavirus 16
  MISC_FEATURE: AAA91663.1 E6 Variant
MFQDPQERPRKLPHLCTELQTTIHDIILECVYCKQQLLRREVYDFAFRDLCIVYRDGNPYAVCDKCLKFYSKISEYRYYCYSVYGTTLEQQYNKPLCDLLIRCINCQKPLCPEEKQRHLDKKQRFHNIRGRWTGRCMSCCRSSRTRRETQL

SEQ ID NO: 43 - protein, 151 aa, Human papillomavirus 16; identical to SEQ ID NO: 42
  MISC_FEATURE: AAA91659.1 E6 Variant

SEQ ID NO: 44 - protein, 151 aa, Human papillomavirus 16; identical to SEQ ID NO: 42
  MISC_FEATURE: AAA91654.1 E6 Variant

SEQ ID NO: 45 - protein, 151 aa, Human papillomavirus 16; identical to SEQ ID NO: 42
  MISC_FEATURE: AAA91666.1 E6 Variant

SEQ ID NO: 46 - protein, 151 aa, Human papillomavirus 16; identical to SEQ ID NO: 42
  MISC_FEATURE: AAA91679.1 E6 Variant

SEQ ID NO: 47 - protein, 151 aa, Human papillomavirus 16; identical to SEQ ID NO: 42
  MISC_FEATURE: AAA91655.1 E6 Variant

SEQ ID NO: 48 - protein, 147 aa, Human papillomavirus 18
  MISC_FEATURE: AHZ96678.1 E6 Variant
MARFEDPTRRPYKLPDLCTELNTSLQDIEITCVYCKTVLELTEVFEFAFKDLFVVYRDSIPHAACHKCIDFYSRIRELRYYSDSVYGDTLEKLTNTGLYNLLIRCLRCQKPLNPAEKLRHLNEKRRFHKIAGHYRGQCHSCCNRARQ

SEQ ID NO: 49 - protein, 158 aa, Human papillomavirus 18; identical to SEQ ID NO: 4
  MISC_FEATURE: ABP99784.1 E6 Variant

SEQ ID NO: 50 - protein, 158 aa, Human papillomavirus 18
  MISC_FEATURE: CAB53096.1 E6 Variant
MARFEDPTRRPYKLPDLCTELNTSLQDIEITCVYCKTVLELTEVFEFAFKDLFVVYRDSIPHAACHKCIDFYSRIRELRHYSDSVYGDTLEKLTNTGLYNLLIRCLRCQKPLNPAEKLRHLNEKRRFHKIAGHYRGQCHSCCNRARQERLQRRRETQV

SEQ ID NO: 51 - protein, 158 aa, Human papillomavirus 18
  MISC_FEATURE: AGU90327.1 E6 Variant
MARFEDPTRRPYKLPDLCTELNTSLQDIEITCVYCKTVLELTEVFEFAFKDLFVVYRDSIPHAACHKCIDFYSRIRELRHYSDSVYGDTLEKLTNTGLYNLLIRCLRCQKPLNPAEKLRHLNEKRRFHKIAGHYRGQCHSCCNQARQERLQRRRETQV

SEQ ID NO: 52 - protein, 158 aa, Human papillomavirus 18
  MISC_FEATURE: ADC35660.1 E6 Variant
MARFEDPTRRPYKVPDLCTELNTSLQDIEITCVYCKTVLELTEVFEFAFKDLFVVYRDSIPHAACHKCIDFYSRIRELRHYSDSVYGDTLEKLTNTGLYNLLIRCLRCQKPLNPAEKLRHLNEKRRFHNIAGHYRGQCHSCCNRARQERLQRRRETQV

SEQ ID NO: 53 - protein, 158 aa, Human papillomavirus 18
  MISC_FEATURE: AHZ96677.1 E6 Variant
MARFEDPTRRPYKLPDLCTELNTSLQDIEITCVYCKTVLELTEVFEFAFKDLFVVYRDSIPHAACHKCIDFYSRIRELRHYSDSVYGDTLEKLTNTGLYNLLIRCLRCQKPLNPAEKLRHLNEKRRFHNIAGHYRGQCHSCCNRARQERLQRHRETQV

SEQ ID NO: 54 - protein, 158 aa, Human papillomavirus 18
  MISC_FEATURE: ABP99736.1 E6 Variant
MARFEDPTRRPYKLPDLCTELNTSLQDIEITCVYCKTVLELTGVFEFAFKDLFVVYRDSIPHAACHKCIDFYSRIRELRHYSDSVYGDTLEKLTNTGLYNLLIRCLRCQKPLNPAEKLRHLNEKRRFHNIAGHYRGQCHSCCNRARQERLQRRRETQV

SEQ ID NO: 55 - protein, 158 aa, Human papillomavirus 18
  MISC_FEATURE: ABP99704.1 E6 Variant
MARFEDPTRRPYKLPDLCTELNTSLQDIEITCVYCKTVLELTEVFEFAFKDLFVVYRDSIPHAACHKCIDFYSRIRELRHYSDSVYGDTLEKLTNTGLYNLLIRCLRCQKPLNPAEKLRHLNEKRRFHNIAGRYRGQCHSCCNRARQERLQRRRETQV

SEQ ID NO: 56 - protein, 90 aa, Human papillomavirus 16
  MISC_FEATURE: ABL96587.1 E7 Variant
MHGDTPTLHEYMLDLQPETTDLYCYEQLSDSSEEEDEIDGPAGQAEPDRAHYNIVTFCCKCDSTLRLCVRSTHVDIRTLEDLLMGTLGIV

SEQ ID NO: 57 - protein, 90 aa, Human papillomavirus 16
  MISC_FEATURE: ABL96591.1 E7 Variant
MHGDTPTLHEYMLDLQPETTDLYCYEQLSDSSEEEDEIDGPAGQAEPDRAHYNIVTFCCKCDSTLRLCVQSTHVDICTLEDLLMGTLGIV

SEQ ID NO: 58 - protein, 92 aa, Human papillomavirus 16
  MISC_FEATURE: AFJ19726.1 E7 Variant
MHGDTPTLHEYMLDLQPETTDLYCYEQLNDSSVEEDEIDGPAGQAEPDRAHYNIVTFCCKCDSTLRLCVQSTHVDIRTLEDLLMGTLGIVCP

SEQ ID NO: 59 - protein, 92 aa, Human papillomavirus 16
  MISC_FEATURE: AFJ19722.1 E7 Variant
MHGDTPTLHEYMLDLQPETTDLYCYEQLNDSSEEVDEIDGPAGQAEPDRAHYNIVTFCCKCDSTLRLCVQSTHVDIRTLEDLLMGTLGIVCP

SEQ ID NO: 60 - protein, 92 aa, Human papillomavirus 16
  MISC_FEATURE: AFJ19752.1 E7 Variant
MHGDTPTLHEYMLDLQPETTDLYCYEQLNDSSEEEDEIDGPAGQAETDRAHYNIVTFCCKCDSTLRLCVQSTHVDIRTLEDLLMGTLGIVCP

SEQ ID NO: 61 - protein, 92 aa, Human papillomavirus 16
  MISC_FEATURE: AFJ19732.1 E7 Variant
MHGDTPTLHEYMLDLQPETTDLYCYEQLKDSSEEEDEVDGPAGQAEPDRAHYNIVTFCCKCDSTLRLCVQSTHVDIRTLEDLLMGTLGIVCP

SEQ ID NO: 62 - protein, 92 aa, Human papillomavirus 16
  MISC_FEATURE: AFJ19762.1 E7 Variant
MHGDTPTLHEYMLDLQPETTDLYCYEQLNDSSEEEDEIDGPAGQAEPDRAHYNIVTFRCKCDSTLRLCVQSTHVDIRTLEDLLMGTLGIVCP

SEQ ID NO: 63 - protein, 92 aa, Human papillomavirus 16
  MISC_FEATURE: AFJ19668.1 E7 Variant
MHGDTPTLHEYMLDLQPETTDLYCYEQLSDSSEEEDEIDGPAGQAEPDRAHYNIVTFCCKCDSTLRLCVQSTHVDIRMLEDLLMGTLGIVCP

SEQ ID NO: 64 - protein, 92 aa, Human papillomavirus 16
  MISC_FEATURE: AFJ19664.1 E7 Variant
MHGDTPTLHEYMLDLQPETTDLYCYEQLSDSSEEEDEIDGPAGQAEPDRAHYNIVTFCCKCDSTLRLCVQSTHVDIRTLEDLLMSTLGIVCP

SEQ ID NO: 65 - protein, 92 aa, Human papillomavirus 16
  MISC_FEATURE: AFJ19766.1 E7 Variant
MHGDTPTLHEYMLDLQPETNDLYCYEQLNDSSEEEDEIDGPAGQAEPDRAHYNIVTFCCKCDFTLRLCVQSTHVDIRTLEDLLMGTLGIVCP

SEQ ID NO: 66 - protein, 92 aa, Human papillomavirus 16
  MISC_FEATURE: AFJ19756.1 E7 Variant
MHGDTPTLHEYMLDLQPETTDLYCYEQLNDSSEEEDEKDGPAGQAEPDRAHYNIVTFCCKCDSTLRLCVQSTHVDIRTLEDLLIGTLGIVCP

SEQ ID NO: 67 - protein, 92 aa, Human papillomavirus 16
  MISC_FEATURE: AFJ19680.1 E7 Variant
MHGDTPTLHEYKLDLQPETTDLYCYEQLNDSSEEEDEIDGPTGQAEPDRAHYNIVTFCCKCDSTLRLCVQSTHVDIRTLEDLLMGTLGIVCP

SEQ ID NO: 68 - protein, 92 aa, Human papillomavirus 16
  MISC_FEATURE: AFJ19772.1 E7 Variant
MHGDTPTLHEYMLDLQPETTDLYCYEQLNDSSEEDDEIDGPAGQAEPDRAHYNIVTFCCKCDSTLRLCVQSTHVDIRTLEDLLMDTLGIVCP

SEQ ID NO: 69 - protein, 92 aa, Human papillomavirus 16
  MISC_FEATURE: AFJ19696.1 E7 Variant
MHGDTPTLHEYKLDLQPETTDLYCYEQLNDSSEEEDEIDGPAGQAEPDRAHYNIVTFCCKCDSTLRLCVQSTHVDIRTLEDLLKGTLGIVCP

SEQ ID NO: 70 - protein, 92 aa, Human papillomavirus 16
  MISC_FEATURE: AFJ19690.1 E7 Variant
MHGDTPTLHEYMLVLQPETTDLYCYEQLNDSSEEEDEIDGPAGQAEPDRAHYNIVTFCCKCDSTLRLCVQSTHVDIRTLEGLLMGTLGIVCP

SEQ ID NO: 71 - protein, 92 aa, Human papillomavirus 16
  MISC_FEATURE: AFJ19712.1 E7 Variant
MHGDTPTLHEYKLDLQPETTDLHCYEQLNDSSEEEDEIDGPAGQAEPDRAHYNIITFCCRCDSTLRLCVQSTHVDIRTLEDLLMGTLGIVCP

SEQ ID NO: 72 - protein, 92 aa, Human papillomavirus 16
  MISC_FEATURE: AGO04504.1 E7 Variant
MHGDTPTLHEYMLGLQPETTDLYCYEQLNDSSEEEDEIDGPAGQAEPDRAHYNIVTFCCMCDSTLRLCVQSTHVDIRTLEDLLMGALGIVCP

SEQ ID NO: 73 - protein, 92 aa, Human papillomavirus 16
  MISC_FEATURE: AFJ19770.1 E7 Variant
MHGDTPTLHEYMLDLQPETTDLYCYEQLYDSSEEEDEIDGPAGQAEPDRAHYNIVTFCCKCDSTLRLCVQSTHVDIQTLEDLLMGALGIVCP

SEQ ID NO: 74 - protein, 92 aa, Human papillomavirus 16
  MISC_FEATURE: AFJ19520.2 E7 Variant
MHGDTPTLHKYMLDLQPETTDLYCYEQLNDSSEEEDEIDGPAGQAEPDRAHYNIVTFYCKCDSTLRLCVQSTHVDIRTLEDLLMSTLGIVCP

SEQ ID NO: 75 - protein, 92 aa, Human papillomavirus 16
  MISC_FEATURE: AFJ19708.1 E7 Variant
MHGDTPKLHEYMLDLQPETTDLYCYEQLNDSSEEEDEIDGQAGQAKPDRAHYNIVTFCCKCDSTLRLCVQSTHVDIRTLEGLLMGTLGIVCP

SEQ ID NO: 76 - protein, 92 aa, Human papillomavirus 16
  MISC_FEATURE: AFJ19674.1 E7 Variant
MHGDTPTLHEYMLDLQPETTDLYCYEQLNDNSEEDHEIDGPDGQAEPDRAHYNIVTFCCKCDSTLRLCVQSTHVDIRTLEDLLMGTLGIVCP

SEQ ID NO: 77 - protein, 92 aa, Human papillomavirus 16
  MISC_FEATURE: AGO04498.1 E7 Variant
MHGDTSTLHEYMLDLQPETTDLYCYEQLNDSSEEEDEIDGPAGQAEPDRAHYNNVTFCCKCDSTLRLCVQSTLVDIRTLEDMLMGTLGIVSP

SEQ ID NO: 78 - protein, 92 aa, Human papillomavirus 16
  MISC_FEATURE: AGO04496.1 E7 Variant
MHGDTPTLHEYVLGLQPETTDLYCYEQLNDSSEEEDEIDGPAGQAEPVRAHYNIVTFCCKCDSTLRFCVQSTRLDIRTLEDLLMGTLGIVCP

SEQ ID NO: 79 - protein, 92 aa, Human papillomavirus 16
  MISC_FEATURE: AFJ19684.1 E7 Variant
MHGDTPTLHEYKLDLQPETTDLYCYEHLNDSSEEEDEIDCPAGQAEPDRAHYKIVTFCCKCDSTLRLCVQSTHVDIRTLEDLLMGILGIVCP

SEQ ID NO: 80 - protein, 92 aa, Human papillomavirus 16
  MISC_FEATURE: AFJ19678.1 E7 Variant
MHGDTPTLHEYKLDLQPETTDLCCYEQLNDSSEEEDEIDGPTGQAEPDRAHYTIVTFCCMCDSTLRLCVQSTHVDIRTLEDLLMGTLGIVCP

SEQ ID NO: 81 - protein, 92 aa, Human papillomavirus 16
  MISC_FEATURE: AFJ19698.1 E7 Variant
MHGDTPTLHEYKLDLQPETTDLYCYEQLNHSSEGEDEIDGPAGQAEPDRAHYNIVTFCCKCDSTPRLCVQSTHVDIRTLEDLLMDTLGIVCP

SEQ ID NO: 82 - protein, 92 aa, Human papillomavirus 16
  MISC_FEATURE: AFJ19746.1 E7 Variant
MHGDTPTLHEYKLDLQPETTDLYCDEQLNHSSEGEDEIDGPAGQAEPDRAHYNIVTFCCKCDSTPRLCVQSTHVDIRTLEDLLMGTLGIVCP

SEQ ID NO: 83 - protein, 93 aa, Human papillomavirus 16
  MISC_FEATURE: AAF13395.1 E7 Variant
MHGDTPTLHEYMLDLQPETTDLYCYEQFNDSSEEEDEIDGPAGQAEPDRAHYNIVTFCCKCDSTLRLCVQSTHVDIRTLEDLLMGTLGIVCPI

SEQ ID NO: 84 - protein, 95 aa, Human papillomavirus 16
  MISC_FEATURE: AFU06654.1 E7 Variant
MHGDTPTLHEYMLDLQPETTDLYCYEQLNDSSEEEDEIDGPAGQAEPDRAHYNIVTFCCKCDSTLRLCVQSTHVDIRTLEDLLMGTLGIVCPICS

SEQ ID NO: 85 - protein, 95 aa, Human papillomavirus 16
  MISC_FEATURE: AFU06650.1 E7 Variant
MHGDTPTLHEYMLDLQPETTDLYCYEQFNDSSEEEDEIDGPAGQAEPDRAHYNIVTFCCKCDSTLRLCVQSTHVDIRTLEDLLMGTLGIVCPICS

SEQ ID NO: 86 - protein, 98 aa, Human papillomavirus 16
  MISC_FEATURE: AAB70738.1 E7 Variant
MHGDTPTLHEYMLDLQPETTDLYCYEQFNDSSEEEDEIDGPAGQAEPDRAHYNIVTFCCKCDSTLRLCVQSTHVDIRTLEDLLMGTLGIVCPICSQKP

SEQ ID NO: 87 - protein, 98 aa, Human papillomavirus 16
  MISC_FEATURE: ACN22555.1 E7 Variant
MHGDTPTLHEYMLDVQPETTDLYCYEQLNDSSEEEDEIDGPAGQAEPDRAHYNIVTFCCKCDSTLRLCVQSTHVDIRTLEDLLMGTLGIVCPICSQKP

SEQ ID NO: 88 - protein, 98 aa, Human papillomavirus 16
  MISC_FEATURE: ABK32510.1 E7 Variant
MHGDTPTLHEYMLDLQPETSDLYCYEQLNDSSEEEDEIDGPAGQAEPDRAHYNIVTFCCKCDSTLRLCVQSTHVDIRTLEDLLMGTLGIVCPICSQKP

SEQ ID NO: 89 - protein, 98 aa, Human papillomavirus 16
  MISC_FEATURE: ABC54573.1 E7 Variant
MHGDTPTLHEYMLDLQPETTDLYCYEQLNDSSEEEDEIDGPAGQAEPDRAHYNIVTFCCKCDSTLRLCVQSTHVDIRALEDLLMGTLGIVCPICSQKP

SEQ ID NO: 90 - protein, 98 aa, Human papillomavirus 16
  MISC_FEATURE: ACN22554.1 E7 Variant
MHGDTPTLHEYMLDLQPETTDLYCYEQLNDRSEEEDEIDGPAGQAEPDRAHYNIVTFCCKCDSTLRLCVQSTHVDIRTLEDLLMGTLGIVCPICSQKP

SEQ ID NO: 91 - protein, 98 aa, Human papillomavirus 16
  MISC_FEATURE: ABK32511.1 E7 Variant
MHGDTPTLHEYMLDLQPETTDLYCYEQLNDSSEEEDEIDGPAGQAKPDRAHYNIVTFCCKCDSTLRLCVQSTHVDISTLEDLLMGTLGIVCPICSQKP

SEQ ID NO: 92 - protein, 98 aa, Human papillomavirus 16
  MISC_FEATURE: ACQ90216.1 E7 Variant
MHGDTPTLHEYMLDLQPETTDLYCYEQLNDSSEEEDEIDGPAGQAEPDRAHYNIVTFRCKCDSTLRLCVQSTHVDIRTLEDLLMGTLGIVCPICSQKP

SEQ ID NO: 93 - protein, 98 aa, Human papillomavirus 16
  MISC_FEATURE: ADY75576.1 E7 Variant
MHGDTPTLHEYMLDLQPETNDLYCYEQLNDSSEEEDEIDGPAGQAEPDRAHYNIVTFCCKCDFTLRLCVQSTHVDIRTLEDLLMGTLGIVCPICSQKP

SEQ ID NO: 94 - protein, 98 aa, Human papillomavirus 16
  MISC_FEATURE: AAM03025.1 E7 Variant
MHGDTPTLHEYMLDLQPETTDLYCYEQLNDSSEEEDEIDGPAGQAEPDRAHYNIVTFCCKCDSTLRLCVQSTHVDICTLEDLLMGTLGIVCPICSQKP

SEQ ID NO: 95 - protein, 98 aa, Human papillomavirus 16
  MISC_FEATURE: AAL96634.1 E7 Variant
MHGDTPTLHEYMLDLQPETTDLYCYEQLSDSSEEEDEIDGPAGQAEPDRAHYNIVTFCCKCDSTLWLCVQSTHVDIRTLEDLLMGTLGIVCPICSQKP

SEQ ID NO: 96 - protein, 105 aa, Human papillomavirus 18; identical to SEQ ID NO: 8
  MISC_FEATURE: ABP99785.1 E7 Variant

SEQ ID NO: 97 - protein, 105 aa, Human papillomavirus 18
  MISC_FEATURE: AGU90416.1 E7 Variant
MYGPKATLQDIVLHLEPQNEIPVDLLCHEQLSDSEEENDEIDGVNHQHLPARRAEPQRHTMLCMCCKCEARIELVVESSADDLRAFQQLFLNTLSFVCPWCASQQ

SEQ ID NO: 98 - protein, 105 aa, Human papillomavirus 18
  MISC_FEATURE: AGU90384.1 E7 Variant
MYGPKATLQDIVLHLEPQNDIPVDLLCHEQLSDSEEENDEIDGVNHQHLPARRAEPQRHTMLCMCCKCEARIELVVESSADDLRAFQQLFLSTLSFVCPWCASQQ

SEQ ID NO: 99 - protein, 105 aa, Human papillomavirus 18
  MISC_FEATURE: CAB53097.1 E7 Variant
MHGPKATLQDIVLHLEPQNEIPVDLLCHEQLSDSEEENDEIDGVNHQHLPARRAEPQRHTMLCMCCKCEARIELVVESSADDLRAFQQLFLKTLSFVCPWCASQQ

SEQ ID NO: 100 - protein, 105 aa, Human papillomavirus 18
  MISC_FEATURE: P06788.2 E7 Variant
MHGPKATLQDIVLHLEPQNEIPVDLLCHEQLSDSEEENDEIDGVNHQHLPARRAEPQRHTMLCMCCKCEARIKLVVESSADDLRAFQQLFLNTLSFVCPWCASQQ

SEQ ID NO: 101 - protein, 105 aa, Human papillomavirus 18
  MISC_FEATURE: CAB53098.1 E7 Variant
MHGPKATLQNIVLHLEPQNEIPVDLLCHEQLSDSEEENDEIDGVNHQHLPARRAEPQRHTMLCMCCKCEARIELVVESSADDLRAFQQLFLKTLSFVCPWCASQQ

SEQ ID NO: 102 - protein, 105 aa, Human papillomavirus 18
  MISC_FEATURE: CAB53099.1 E7 Variant
MHGPKATLQDIVLHLEPQNEIPVGLLCHEQLSDSEEENDEIDGVNHQHLPARRAEPQRHTMLCMCCKCEARIELVVESSADDLRAFQQLFLKTLSFVCPWCASQQ

SEQ ID NO: 103 - protein, 145 aa, Human papillomavirus 18
  MISC_FEATURE: AGM34425.1 E6 Variant
LPDLCTELNTSLQDIEITCVYCKTVLELTEVFEFAFKDLFVVYRDSIPHAACHKCIDFYSRIRELRYYSDSVYGDTLEKLTNTGLYNLLIRCLRCQKPLNPAEKLRHLNEKRRFHKIAGHYRGQCHSCCNRARQERLQRRRETQV

SEQ ID NO: 104 - protein, 145 aa, Human papillomavirus 18
  MISC_FEATURE: AGM34424.1 E6 Variant
LPDLCTELNTSLQDIEITCVYCKTVLELTEVFEFAFKDLFVVYRDSIPHAACHKCIDFYSRIRELRHYSDSVYGDTLEKLTNTGLYNLLIRCLRCQKPLNPAEKLRHLNEKRRFHNIAGHYRGQCHSCCNRARQERLQRRRETQV

SEQ ID NO: 105 - DNA, 6085 bp, Artificial Sequence
  C-1 mutant
  misc_feature (1368)..(1433): encodes tPA
  misc_feature (1434)..(1925): encodes FLT3L
  misc_feature (1932)..(2186): 16E6N (H21Q)
  misc_feature (1932)..(2789): 16E6/E7
  misc_feature (2187)..(2381): 16E7N
  misc_feature (2382)..(2645): 16E6C (Y85H, V90L)
  misc_feature (2646)..(2789): 16E7C
  misc_feature (2790)..(3671): 18E6/E7
taccgatgtacgggccagatatacgcgttgacattgattattgactagttattaatagtaatcaattacggggtcattagttcatagcccatatatggagttccgcgttacataacttacggtaaatggcccgcctggctgaccgcccaacgacccccgcccattgacgtcaataatgacgtatgttcccatagtaacgccaatagggactttccattgacgtcaatgggtggagtatttacggtaaactgcccacttggcagtacatcaagtgtatcatatgccaagtacgccccctattgacgtcaatgacggtaaatggcccgcctggcattatgcccagtacatgaccttatgggactttcctacttggcagtacatctacgtattagtcatcgctattaccatggtgatgcggttttggcagtacatcaatgggcgtggatagcggtttgactcacggggatttccaagtctccaccccattgacgtcaatgggagtttgttttggcaccaaaatcaacgggactttccaaaatgtcgtaacaactccgccccattgacgcaaatgggcggtaggcgtgtacggtgggaggtctatataagcagagctctctggctaactagagaacccactgcttactggcttatcgaaattaatacgactcactatagggagacccaagctggctagcgtgagtttggggacccttgattgttctttctttttcgctattgtaaaattcatgttatatggagggggcaaagttttcagggtgttgtttagaacgggaagatgtcccttgtatcaccatggaccctcatgataattttgtttctttcactttctactctgttgacaaccattgtctcctcttattttcttttcattttctgtaactttttcgttaaactttagcttgcatttgtaacgaatttttaaattcacttttgtttatttgtcagattgtaagtactttctctaatcacttttttttcaaggcaatcagggtatattatattgtacttcagcacagttttagagaacaattgttataattaaatgataaggtagaatatttctgcatataaattctggctggcgtggaaatattcttattggtagaaacaactacatcctggtcatcatcctgcctttctctttatggttacaatgatatacactgtttgagatgaggataaaatactctgagtccaaaccgggcccctctgctaaccatgttcatgccttcttctttttcctacagctcctgggcaacgtgctggttattgtgctgtctcatcattttggcaaagaattgtaatacgactcactatagggcgaattgaagcttggtaccgccaccatggatgctatgaaacggggcctgtgctgcgtgctgctcctgtgcggcgctgtgtttgtgagccctagcatcacccaggactgctccttccaacacagccccatctcctccgacttcgctgtcaaaatccgtgagctgtctgactacctgcttcaagattacccagtcaccgtggcctccaacctgcaggacgaggagctctgcgggggcctctggcggctggtcctggcacagcgctggatggagcggctcaagactgtcgctgggtccaagatgcaaggcttgctggagcgcgtgaacacggagatacactttgtcaccaaatgtgcctttcagcccccccccagctgtcttcgcttcgtccagaccaacatctcccgcctcctgcaggagacctccgagcagctggtggcgctgaagccctggatcactcgccagaacttctcccggtgcctggagctgcagtgtcagcccgactcctcaaccctgccacccccatggagtccccggcccctggaggccacagccccgacagccccgggcggcggcagcggcgatgctagcatgcaccagaagagaaccgccatgttccaggaccctcaggagagacctaggaagctgcctcagctgtgtacagagctccagacaaccatccacgacatcatcctggagtgcgtgtactgtaagcagcagctgctgagaagagaggtgtacgacttcgccttcagagacctgtgcatcgtgtacagagacggcaacccttacgccgtgtgcgataagtgtctgaagttctattccaaaatctccgaatataggtacatgcacggcgacacccctaccctgcacgagtacatgctggacctccagcctgagaccacagacctgtactgctacgagcagctgaacgacagctctgaggaagaggacgagattgacggacctgctggccaggccgagcctgacagagcccactacaatatcgtgacattctgttgcaaatgcgactccacactggacaagtgcctgaagttctacagcaagatctctgagtacagacactactgctactctctgtacggcaccacactggagcagcagtacaacaagcctctgtgcgacctcctgatccgctgcatcaactgccagaagcctctgtgccctgaggagaagcagagacacctggacaagaagcagcggttccacaacatcagaggcagatggaccggcaggtgcatgtcctgctgtagatcctccagaaccagacgggagacccagctgcactacaacatcgtgaccttctgctgcaagtgcgactctaccctgagactgtgcgtgcagtctacccacgtggacatcagaaccctggaggacctgctgatgggcaccctgggcatcgtgtgccctatctgctctcagaagcctatggccaggttcgaggaccctaccagaagaccctacaagctgcctgacctgtgcaccgagctgaacacctctctgcaagacatcgagatcacctgcgtgtactgcaagaccgtgctggagctgaccgaggtgttcgagttcgccttcaaggacctgttcgtggtgtacagagacagcatccctcacgctgcctgccacaagtgcatcgacttctattccaggatcagggagctgcgctattactccgactctgtgatgtacggccccaaggccaccctccaggacatcgtgctgcacctggagcctcagaacgagatccccgtggacctgctgtgccacgagcagctgtctgactctgaagaggagaacgacgagatcgacggcgtgaaccaccagcacctgcctgccaggagagctgaaccccagcggcataccatgctgtgtatgtgcttctactctaggatcagagagctgaggtactactctgactctgtgtacggcgacaccctggagaagctgaccaacaccggcctgtacaacctgctgatccggtgcctgaggtgccagaagcctctgaaccctgccgagaagctgagacacctgaacgagaagagaagattccacaagatcgctggccactacagaggccagtgccactcttgctgcaacagagccagacaggagagactccagcggagaagggagacccaggtggccagaagagccgagcctcagagacacaccatgctgtgcatgtgctgcaagtgcgaggccagaatcgagctggtggtggagagctctgccgacgacctgagagccttccagcagctgttcctgtctaccctgagcttcgtgtgcccttggtgcgcctctcagcagtaatctagagtcggggcggccggccgcttcgagcagacatgataagatacattgatgagtttggacaaaccacaactagaatgcagtgaaaaaaatgctttatttgtgaaatttgtgatgctattgctttatttgtaaccattataagctgcaataaacaagttaacaacaacaattgcattcattttatgtttcaggttcagggggaggtgtgggaggttttttaaagcaagtaaaacctctacaaatgtggtaaaatcgataaggatctgaacgatggagcggagaatgggcggaactgggcggagttaggggcgggatgggcggagttaggggcgggactatggttgctgactaattgagatgcatgctttgcatacttctgcctgctggggagcctggggactttccacacctggttgctgactaattgagatgcatgctttgcatacttctgcctgctggggagcctggggactttccacaccctaactgacacacattccacagcggatccgtcgacttcagaagaactcgtcaagaaggcgatagaaggcgatgcgccgcgaatcgggagcggcgataccgtagagcacgaggaagcggtcagcccattcgccgccaagctcttcagcaatatcacgggtagccaacgctatgtcctgatagcggtccgccacacccagccggccacagtcgatgaatccagaaaagcggccattttccaccatgatattcggcaagcaggcatcgccatgggtcacgacgagatcctcgccgtcgggcatgctcgccttgagcctggcgaacagttcggctggcgcgagcccctgatgctcttcgtccagatcatcctgatcgacaagaccggcttccatccgagtacgtgctcgctcgatgcgatgtttcgcttggtggtcgaatgggcaggtagccggatcaagcgtatgcagccgccgcattgcatcagccatgatggatactttctcggcaggagcaaggtgagatgacaggagatcctgccccggcacttcgcccaatagcagccagtcccttcccgcttcagtgacaacgtcgagcacagctgcgcaaggaacgcccgtcgtggccagccacgatagccgcgctgcctcgtcttgcagttcattcagggcaccggacaggtcggtcttgacaaaaagaaccgggcgcccctgcgctgacagccggaacacggcggcatcagagcagccgattgtctgttgtgcccagtcatagccgaatagcctctccacccaagcggccggagaacctgcgtgcaatccatcttgttcaatcatgcgaaacgatcctcatcctgtctcttgatcagatcttgatcccctgcgccatcagatccttggcggcaagaaagccatccagtttactttgcagggcttcccaaccttaccagagggcgccccagctggcaattccggttcgcttgctgtccataaaaccgcccagtctagctatcgccatgtaagcccactgcaagctacctgctttctctttgcgcttgcgttttcccttgtccagatagcccagtagctgacattcatccggggtcagcaccgtttctgcggactggctttctacgtgaaaaggatctaggtgaagatcctttttgataatctcatgaccaaaatcccttaacgtgagttttcgttccactgagcgtcagaccccgtagaaaagatcaaaggatcttcttgagatcctttttttctgcgcgtaatctgctgcttgcaaacaaaaaaaccaccgctaccagcggtggtttgtttgccggatcaagagctaccaactctttttccgaaggtaactggcttcagcagagcgcagataccaaatactgttcttctagtgtagccgtagttaggccaccacttcaagaactctgtagcaccgcctacatacctcgctctgctaatcctgttaccagtggctgctgccagtggcgataagtcgtgtcttaccgggttggactcaagacgatagttaccggataaggcgcagcggtcgggctgaacggggggttcgtgcacacagcccagcttggagcgaacgacctacaccgaactgagatacctacagcgtgagctatgagaaagcgccacgcttcccgaagggagaaaggcggacaggtatccggtaagcggcagggtcggaacaggagagcgcacgagggagcttccagggggaaacgcccggtatctttatagtcctgtcgggtttcgccacctctgacttgagcgtcgatttttgtgatgctcgtcaggggggcggagcctatggaaaaacgccagcaacgcggcctttttacggttcctggccttttgctggccttttgctcacatgttcgggcccaatcgacccgggcgacggccagtgaattg

SEQ ID NO: 106 - protein, 767 aa, Artificial Sequence
  C-1
MDAMKRGLCCVLLLCGAVFVSPSITQDCSFQHSPISSDFAVKIRELSDYLLQDYPVTVASNLQDEELCGGLWRLVLAQRWMERLKTVAGSKMQGLLERVNTEIHFVTKCAFQPPPSCLRFVQTNISRLLQETSEQLVALKPWITRQNFSRCLELQCQPDSSTLPPPWSPRPLEATAPTAPGGGSGDASMHQKRTAMFQDPQERPRKLPQLCTELQTTIHDIILECVYCKQQLLRREVYDFAFRDLCIVYRDGNPYAVCDKCLKFYSKISEYRYMHGDTPTLHEYMLDLQPETTDLYCYEQLNDSSEEEDEIDGPAGQAEPDRAHYNIVTFCCKCDSTLDKCLKFYSKISEYRHYCYSLYGTTLEQQYNKPLCDLLIRCINCQKPLCPEEKQRHLDKKQRFHNIRGRWTGRCMSCCRSSRTRRETQLHYNIVTFCCKCDSTLRLCVQSTHVDIRTLEDLLMGTLGIVCPICSQKPMARFEDPTRRPYKLPDLCTELNTSLQDIEITCVYCKTVLELTEVFEFAFKDLFVVYRDSIPHAACHKCIDFYSRIRELRYYSDSVMYGPKATLQDIVLHLEPQNEIPVDLLCHEQLSDSEEENDEIDGVNHQHLPARRAEPQRHTMLCMCFYSRIRELRYYSDSVYGDTLEKLTNTGLYNLLIRCLRCQKPLNPAEKLRHLNEKRRFHKIAGHYRGQCHSCCNRARQERLQRRRETQVARRAEPQRHTMLCMCCKCEARIELVVESSADDLRAFQQLFLSTLSFVCPWCASQQ

SEQ ID NO: 107 - DNA, 6085 bp, Artificial Sequence
  C-2 mutant
  misc_feature (1368)..(1433): encodes tPA
  misc_feature (1434)..(1925): encodes FLT3L
  misc_feature (1932)..(2186): 16E6N
  misc_feature (1932)..(2789): 16E6/E7
  misc_feature (2187)..(2381): 16E7N (M12K, N29S)
  misc_feature (2382)..(2645): 16E6C
  misc_feature (2646)..(2789): 16E7C (R77S, G85S)
  misc_feature (2790)..(3671): 18E6/E7
taccgatgtacgggccagatatacgcgttgacattgattattgactagttattaatagtaatcaattacggggtcattagttcatagcccatatatggagttccgcgttacataacttacggtaaatggcccgcctggctgaccgcccaacgacccccgcccattgacgtcaataatgacgtatgttcccatagtaacgccaatagggactttccattgacgtcaatgggtggagtatttacggtaaactgcccacttggcagtacatcaagtgtatcatatgccaagtacgccccctattgacgtcaatgacggtaaatggcccgcctggcattatgcccagtacatgaccttatgggactttcctacttggcagtacatctacgtattagtcatcgctattaccatggtgatgcggttttggcagtacatcaatgggcgtggatagcggtttgactcacggggatttccaagtctccaccccattgacgtcaatgggagtttgttttggcaccaaaatcaacgggactttccaaaatgtcgtaacaactccgccccattgacgcaaatgggcggtaggcgtgtacggtgggaggtctatataagcagagctctctggctaactagagaacccactgcttactggcttatcgaaattaatacgactcactatagggagacccaagctggctagcgtgagtttggggacccttgattgttctttctttttcgctattgtaaaattcatgttatatggagggggcaaagttttcagggtgttgtttagaacgggaagatgtcccttgtatcaccatggaccctcatgataattttgtttctttcactttctactctgttgacaaccattgtctcctcttattttcttttcattttctgtaactttttcgttaaactttagcttgcatttgtaacgaatttttaaattcacttttgtttatttgtcagattgtaagtactttctctaatcacttttttttcaaggcaatcagggtatattatattgtacttcagcacagttttagagaacaattgttataattaaatgataaggtagaatatttctgcatataaattctggctggcgtggaaatattcttattggtagaaacaactacatcctggtcatcatcctgcctttctctttatggttacaatgatatacactgtttgagatgaggataaaatactctgagtccaaaccgggcccctctgctaaccatgttcatgccttcttctttttcctacagctcctgggcaacgtgctggttattgtgctgtctcatcattttggcaaagaattgtaatacgactcactatagggcgaattgaagcttggtaccgccaccatggatgctatgaaacggggcctgtgctgcgtgctgctcctgtgcggcgctgtgtttgtgagccctagcatcacccaggactgctccttccaacacagccccatctcctccgacttcgctgtcaaaatccgtgagctgtctgactacctgcttcaagattacccagtcaccgtggcctccaacctgcaggacgaggagctctgcgggggcctctggcggctggtcctggcacagcgctggatggagcggctcaagactgtcgctgggtccaagatgcaaggcttgctggagcgcgtgaacacggagatacactttgtcaccaaatgtgcctttcagcccccccccagctgtcttcgcttcgtccagaccaacatctcccgcctcctgcaggagacctccgagcagctggtggcgctgaagccctggatcactcgccagaacttctcccggtgcctggagctgcagtgtcagcccgactcctcaaccctgccacccccatggagtccccggcccctggaggccacagccccgacagccccgggcggcggcagcggcgatgctagcatgcaccagaagagaaccgccatgttccaggaccctcaggagagacctaggaagctgcctcacctgtgtacagagctccagacaaccatccacgacatcatcctggagtgcgtgtactgtaagcagcagctgctgagaagagaggtgtacgacttcgccttcagagacctgtgcatcgtgtacagagacggcaacccttacgccgtgtgcgataagtgtctgaagttctattccaaaatctccgaatataggtacatgcacggcgacacccctaccctgcacgagtacaagctggacctccagcctgagaccacagacctgtactgctacgagcagctgtctgacagctctgaggaagaggacgagattgacggacctgctggccaggccgagcctgacagagcccactacaatatcgtgacattctgttgcaaatgcgactccacactggacaagtgcctgaagttctacagcaagatctctgagtacagatactactgctactctgtgtacggcaccacactggagcagcagtacaacaagcctctgtgcgacctcctgatccgctgcatcaactgccagaagcctctgtgccctgaggagaagcagagacacctggacaagaagcagcggttccacaacatcagaggcagatggaccggcaggtgcatgtcctgctgtagatcctccagaaccagacgggagacccagctgcactacaacatcgtgaccttctgctgcaagtgcgactctaccctgagactgtgcgtgcagtctacccacgtggacatcctcaccctggaggacctgctgatgctcaccctgggcatcgtgtgccctatctgctctcagaagcctatggccaggttcgaggaccctaccagaagaccctacaagctgcctgacctgtgcaccgagctgaacacctctctgcaagacatcgagatcacctgcgtgtactgcaagaccgtgctggagctgaccgaggtgttcgagttcgccttcaaggacctgttcgtggtgtacagagacagcatccctcacgctgcctgccacaagtgcatcgacttctattccaggatcagggagctgcgctattactccgactctgtgatgtacggccccaaggccaccctccaggacatcgtgctgcacctggagcctcagaacgagatccccgtggacctgctgtgccacgagcagctgtctgactctgaagaggagaacgacgagatcgacggcgtgaaccaccagcacctgcctgccaggagagctgaaccccagcggcataccatgctgtgtatgtgcttctactctaggatcagagagctgaggtactactctgactctgtgtacggcgacaccctggagaagctgaccaacaccggcctgtacaacctgctgatccggtgcctgaggtgccagaagcctctgaaccctgccgagaagctgagacacctgaacgagaagagaagattccacaagatcgctggccactacagaggccagtgccactcttgctgcaacagagccagacaggagagactccagcggagaagggagacccaggtggccagaagagccgagcctcagagacacaccatgctgtgcatgtgctgcaagtgcgaggccagaatcgagctggtggtggagagctctgccgacgacctgagagccttccagcagctgttcctgtctaccctgagcttcgtgtgcccttggtgcgcctctcagcagtaatctagagtcggggcggccggccgcttcgagcagacatgataagatacattgatgagtttggacaaaccacaactagaatgcagtgaaaaaaatgctttatttgtgaaatttgtgatgctattgctttatttgtaaccattataagctgcaataaacaagttaacaacaacaattgcattcattttatgtttcaggttcagggggaggtgtgggaggttttttaaagcaagtaaaacctctacaaatgtggtaaaatcgataaggatctgaacgatggagcggagaatgggcggaactgggcggagttaggggcgggatgggcggagttaggggcgggactatggttgctgactaattgagatgcatgctttgcatacttctgcctgctggggagcctggggactttccacacctggttgctgactaattgagatgcatgctttgcatacttctgcctgctggggagcctggggactttccacaccctaactgacacacattccacagcggatccgtcgacttcagaagaactcgtcaagaaggcgatagaaggcgatgcgccgcgaatcgggagcggcgataccgtagagcacgaggaagcggtcagcccattcgccgccaagctcttcagcaatatcacgggtagccaacgctatgtcctgatagcggtccgccacacccagccggccacagtcgatgaatccagaaaagcggccattttccaccatgatattcggcaagcaggcatcgccatgggtcacgacgagatcctcgccgtcgggcatgctcgccttgagcctggcgaacagttcggctggcgcgagcccctgatgctcttcgtccagatcatcctgatcgacaagaccggcttccatccgagtacgtgctcgctcgatgcgatgtttcgcttggtggtcgaatgggcaggtagccggatcaagcgtatgcagccgccgcattgcatcagccatgatggatactttctcggcaggagcaaggtgagatgacaggagatcctgccccggcacttcgcccaatagcagccagtcccttcccgcttcagtgacaacgtcgagcacagctgcgcaaggaacgcccgtcgtggccagccacgatagccgcgctgcctcgtcttgcagttcattcagggcaccggacaggtcggtcttgacaaaaagaaccgggcgcccctgcgctgacagccggaacacggcggcatcagagcagccgattgtctgttgtgcccagtcatagccgaatagcctctccacccaagcggccggagaacctgcgtgcaatccatcttgttcaatcatgcgaaacgatcctcatcctgtctcttgatcagatcttgatcccctgcgccatcagatccttggcggcaagaaagccatccagtttactttgcagggcttcccaaccttaccagagggcgccccagctggcaattccggttcgcttgctgtccataaaaccgcccagtctagctatcgccatgtaagcccactgcaagctacctgctttctctttgcgcttgcgttttcccttgtccagatagcccagtagctgacattcatccggggtcagcaccgtttctgcggactggctttctacgtgaaaaggatctaggtgaagatcctttttgataatctcatgaccaaaatcccttaacgtgagttttcgttccactgagcgtcagaccccgtagaaaagatcaaaggatcttcttgagatcctttttttctgcgcgtaatctgctgcttgcaaacaaaaaaaccaccgctaccagcggtggtttgtttgccggatcaagagctaccaactctttttccgaaggtaactggcttcagcagagcgcagataccaaatactgttcttctagtgtagccgtagttaggccaccacttcaagaactctgtagcaccgcctacatacctcgctctgctaatcctgttaccagtggctgctgccagtggcgataagtcgtgtcttaccgggttggactcaagacgatagttaccggataaggcgcagcggtcgggctgaacggggggttcgtgcacacagcccagcttggagcgaacgacctacaccgaactgagatacctacagcgtgagctatgagaaagcgccacgcttcccgaagggagaaaggcggacaggtatccggtaagcggcagggtcggaacaggagagcgcacgagggagcttccagggggaaacgcccggtatctttatagtcctgtcgggtttcgccacctctgacttgagcgtcgatttttgtgatgctcgtcaggggggcggagcctatggaaaaacgccagcaacgcggcctttttacggttcctggccttttgctggccttttgctcacatgttcgggcccaatcgacccgggcgacggccagtgaattg

SEQ ID NO: 108 - protein, 767 aa, Artificial Sequence
  C-2
MDAMKRGLCCVLLLCGAVFVSPSITQDCSFQHSPISSDFAVKIRELSDYLLQDYPVTVASNLQDEELCGGLWRLVLAQRWMERLKTVAGSKMQGLLERVNTEIHFVTKCAFQPPPSCLRFVQTNISRLLQETSEQLVALKPWITRQNFSRCLELQCQPDSSTLPPPWSPRPLEATAPTAPGGGSGDASMHQKRTAMFQDPQERPRKLPHLCTELQTTIHDIILECVYCKQQLLRREVYDFAFRDLCIVYRDGNPYAVCDKCLKFYSKISEYRYMHGDTPTLHEYKLDLQPETTDLYCYEQLSDSSEEEDEIDGPAGQAEPDRAHYNIVTFCCKCDSTLDKCLKFYSKISEYRYYCYSVYGTTLEQQYNKPLCDLLIRCINCQKPLCPEEKQRHLDKKQRFHNIRGRWTGRCMSCCRSSRTRRETQLHYNIVTFCCKCDSTLRLCVQSTHVDILTLEDLLMLTLGIVCPICSQKPMARFEDPTRRPYKLPDLCTELNTSLQDIEITCVYCKTVLELTEVFEFAFKDLFVVYRDSIPHAACHKCIDFYSRIRELRYYSDSVMYGPKATLQDIVLHLEPQNEIPVDLLCHEQLSDSEEENDEIDGVNHQHLPARRAEPQRHTMLCMCFYSRIRELRYYSDSVYGDTLEKLTNTGLYNLLIRCLRCQKPLNPAEKLRHLNEKRRFHKIAGHYRGQCHSCCNRARQERLQRRRETQVARRAEPQRHTMLCMCCKCEARIELVVESSADDLRAFQQLFLSTLSFVCPWCASQQ

SEQ ID NO: 109 - DNA, 5995 bp, Artificial Sequence
  D-1 (overlapping-1)
  misc_feature (1368)..(1433): encodes tPA
  misc_feature (1434)..(1925): encodes FLT3L
  misc_feature (1932)..(2165): 16E6N (1-78aa)
  misc_feature (2166)..(2339): 16E7N (1-58aa)
  misc_feature (2340)..(2579): 16E6C (79-158aa)
  misc_feature (2580)..(2699): 16E7C (59-98aa)
  misc_feature (2700)..(3581): 18E6/E7
taccgatgtacgggccagatatacgcgttgacattgattattgactagttattaatagtaatcaattacggggtcattagttcatagcccatatatggagttccgcgttacataacttacggtaaatggcccgcctggctgaccgcccaacgacccccgcccattgacgtcaataatgacgtatgttcccatagtaacgccaatagggactttccattgacgtcaatgggtggagtatttacggtaaactgcccacttggcagtacatcaagtgtatcatatgccaagtacgccccctattgacgtcaatgacggtaaatggcccgcctggcattatgcccagtacatgaccttatgggactttcctacttggcagtacatctacgtattagtcatcgctattaccatggtgatgcggttttggcagtacatcaatgggcgtggatagcggtttgactcacggggatttccaagtctccaccccattgacgtcaatgggagtttgttttggcaccaaaatcaacgggactttccaaaatgtcgtaacaactccgccccattgacgcaaatgggcggtaggcgtgtacggtgggaggtctatataagcagagctctctggctaactagagaacccactgcttactggcttatcgaaattaatacgactcactatagggagacccaagctggctagcgtgagtttggggacccttgattgttctttctttttcgctattgtaaaattcatgttatatggagggggcaaagttttcagggtgttgtttagaacgggaagatgtcccttgtatcaccatggaccctcatgataattttgtttctttcactttctactctgttgacaaccattgtctcctcttattttcttttcattttctgtaactttttcgttaaactttagcttgcatttgtaacgaatttttaaattcacttttgtttatttgtcagattgtaagtactttctctaatcacttttttttcaaggcaatcagggtatattatattgtacttcagcacagttttagagaacaattgttataattaaatgataaggtagaatatttctgcatataaattctggctggcgtggaaatattcttattggtagaaacaactacatcctggtcatcatcctgcctttctctttatggttacaatgatatacactgtttgagatgaggataaaatactctgagtccaaaccgggcccctctgctaaccatgttcatgccttcttctttttcctacagctcctgggcaacgtgctggttattgtgctgtctcatcattttggcaaagaattgtaatacgactcactatagggcgaattgaagcttggtaccgccaccatggatgctatgaaacggggcctgtgctgcgtgctgctcctgtgcggcgctgtgtttgtgagccctagcatcacccaggactgctccttccaacacagccccatctcctccgacttcgctgtcaaaatccgtgagctgtctgactacctgcttcaagattacccagtcaccgtggcctccaacctgcaggacgaggagctctgcgggggcctctggcggctggtcctggcacagcgctggatggagcggctcaagactgtcgctgggtccaagatgcaaggcttgctggagcgcgtgaacacggagatacactttgtcaccaaatgtgcctttcagcccccccccagctgtcttcgcttcgtccagaccaacatctcccgcctcctgcaggagacctccgagcagctggtggcgctgaagccctggatcactcgccagaacttctcccggtgcctggagctgcagtgtcagcccgactcctcaaccctgccacccccatggagtccccggcccctggaggccacagccccgacagccccgggcggcggcagcggcgatgctagcatgcaccagaagagaaccgccatgttccaggaccctcaggagagacctaggaagctgcctcacctgtgtacagagctccagacaaccatccacgacatcatcctggagtgcgtgtactgtaagcagcagctgctgagaagagaggtgtacgacttcgccttcagagacctgtgcatcgtgtacagagacggcaacccttacgccgtgtgcgataagtgtctgaagttctattccatgcacggcgacacccctaccctgcacgagtacatgctggacctccagcctgagaccacagacctgtactgctacgagcagctgaacgacagctctgaggaagaggacgagattgacggacctgctggccaggccgagcctgacagagcccactacaatatcgtgacattctgtaagatctctgagtacagatactactgctactctgtgtacggcaccacactggagcagcagtacaacaagcctctgtgcgacctcctgatccgctgcatcaactgccagaagcctctgtgccctgaggagaagcagagacacctggacaagaagcagcggttccacaacatcagaggcagatggaccggcaggtgcatgtcctgctgtagatcctccagaaccagacgggagacccagctgtgcaagtgcgactctaccctgagactgtgcgtgcagtctacccacgtggacatcagaaccctggaggacctgctgatgggcaccctgggcatcgtgtgccctatctgctctcagaagcctatggccaggttcgaggaccctaccagaagaccctacaagctgcctgacctgtgcaccgagctgaacacctctctgcaagacatcgagatcacctgcgtgtactgcaagaccgtgctggagctgaccgaggtgttcgagttcgccttcaaggacctgttcgtggtgtacagagacagcatccctcacgctgcctgccacaagtgcatcgacttctattccaggatcagggagctgcgctattactccgactctgtgatgtacggccccaaggccaccctccaggacatcgtgctgcacctggagcctcagaacgagatccccgtggacctgctgtgccacgagcagctgtctgactctgaagaggagaacgacgagatcgacggcgtgaaccaccagcacctgcctgccaggagagctgaaccccagcggcataccatgctgtgtatgtgcttctactctaggatcagagagctgaggtactactctgactctgtgtacggcgacaccctggagaagctgaccaacaccggcctgtacaacctgctgatccggtgcctgaggtgccagaagcctctgaaccctgccgagaagctgagacacctgaacgagaagagaagattccacaagatcgctggccactacagaggccagtgccactcttgctgcaacagagccagacaggagagactccagcggagaagggagacccaggtggccagaagagccgagcctcagagacacaccatgctgtgcatgtgctgcaagtgcgaggccagaatcgagctggtggtggagagctctgccgacgacctgagagccttccagcagctgttcctgtctaccctgagcttcgtgtgcccttggtgcgcctctcagcagtaatctagagtcggggcggccggccgcttcgagcagacatgataagatacattgatgagtttggacaaaccacaactagaatgcagtgaaaaaaatgctttatttgtgaaatttgtgatgctattgctttatttgtaaccattataagctgcaataaacaagttaacaacaacaattgcattcattttatgtttcaggttcagggggaggtgtgggaggttttttaaagcaagtaaaacctctacaaatgtggtaaaatcgataaggatctgaacgatggagcggagaatgggcggaactgggcggagttaggggcgggatgggcggagttaggggcgggactatggttgctgactaattgagatgcatgctttgcatacttctgcctgctggggagcctggggactttccacacctggttgctgactaattgagatgcatgctttgcatacttctgcctgctggggagcctggggactttccacaccctaactgacacacattccacagcggatccgtcgacttcagaagaactcgtcaagaaggcgatagaaggcgatgcgccgcgaatcgggagcggcgataccgtagagcacgaggaagcggtcagcccattcgccgccaagctcttcagcaatatcacgggtagccaacgctatgtcctgatagcggtccgccacacccagccggccacagtcgatgaatccagaaaagcggccattttccaccatgatattcggcaagcaggcatcgccatgggtcacgacgagatcctcgccgtcgggcatgctcgccttgagcctggcgaacagttcggctggcgcgagcccctgatgctcttcgtccagatcatcctgatcgacaagaccggcttccatccgagtacgtgctcgctcgatgcgatgtttcgcttggtggtcgaatgggcaggtagccggatcaagcgtatgcagccgccgcattgcatcagccatgatggatactttctcggcaggagcaaggtgagatgacaggagatcctgccccggcacttcgcccaatagcagccagtcccttcccgcttcagtgacaacgtcgagcacagctgcgcaaggaacgcccgtcgtggccagccacgatagccgcgctgcctcgtcttgcagttcattcagggcaccggacaggtcggtcttgacaaaaagaaccgggcgcccctgcgctgacagccggaacacggcggcatcagagcagccgattgtctgttgtgcccagtcatagccgaatagcctctccacccaagcggccggagaacctgcgtgcaatccatcttgttcaatcatgcgaaacgatcctcatcctgtctcttgatcagatcttgatcccctgcgccatcagatccttggcggcaagaaagccatccagtttactttgcagggcttcccaaccttaccagagggcgccccagctggcaattccggttcgcttgctgtccataaaaccgcccagtctagctatcgccatgtaagcccactgcaagctacctgctttctctttgcgcttgcgttttcccttgtccagatagcccagtagctgacattcatccggggtcagcaccgtttctgcggactggctttctacgtgaaaaggatctaggtgaagatcctttttgataatctcatgaccaaaatcccttaacgtgagttttcgttccactgagcgtcagaccccgtagaaaagatcaaaggatcttcttgagatcctttttttctgcgcgtaatctgctgcttgcaaacaaaaaaaccaccgctaccagcggtggtttgtttgccggatcaagagctaccaactctttttccgaaggtaactggcttcagcagagcgcagataccaaatactgttcttctagtgtagccgtagttaggccaccacttcaagaactctgtagcaccgcctacatacctcgctctgctaatcctgttaccagtggctgctgccagtggcgataagtcgtgtcttaccgggttggactcaagacgatagttaccggataaggcgcagcggtcgggctgaacggggggttcgtgcacacagcccagcttggagcgaacgacctacaccgaactgagatacctacagcgtgagctatgagaaagcgccacgcttcccgaagggagaaaggcggacaggtatccggtaagcggcagggtcggaacaggagagcgcacgagggagcttccagggggaaacgcccggtatctttatagtcctgtcgggtttcgccacctctgacttgagcgtcgatttttgtgatgctcgtcaggggggcggagcctatggaaaaacgccagcaacgcggcctttttacggttcctggccttttgctggccttttgctcacatgttcgggcccaatcgacccgggcgacggccagtgaattg

SEQ ID NO: 110 - protein, 737 aa, Artificial Sequence
  D-1
MDAMKRGLCCVLLLCGAVFVSPSITQDCSFQHSPISSDFAVKIRELSDYLLQDYPVTVASNLQDEELCGGLWRLVLAQRWMERLKTVAGSKMQGLLERVNTEIHFVTKCAFQPPPSCLRFVQTNISRLLQETSEQLVALKPWITRQNFSRCLELQCQPDSSTLPPPWSPRPLEATAPTAPGGGSGDASMHQKRTAMFQDPQERPRKLPHLCTELQTTIHDIILECVYCKQQLLRREVYDFAFRDLCIVYRDGNPYAVCDKCLKFYSMHGDTPTLHEYMLDLQPETTDLYCYEQLNDSSEEEDEIDGPAGQAEPDRAHYNIVTFCKISEYRYYCYSVYGTTLEQQYNKPLCDLLIRCINCQKPLCPEEKQRHLDKKQRFHNIRGRWTGRCMSCCRSSRTRRETQLCKCDSTLRLCVQSTHVDIRTLEDLLMGTLGIVCPICSQKPMARFEDPTRRPYKLPDLCTELNTSLQDIEITCVYCKTVLELTEVFEFAFKDLFVVYRDSIPHAACHKCIDFYSRIRELRYYSDSVMYGPKATLQDIVLHLEPQNEIPVDLLCHEQLSDSEEENDEIDGVNHQHLPARRAEPQRHTMLCMCFYSRIRELRYYSDSVYGDTLEKLTNTGLYNLLIRCLRCQKPLNPAEKLRHLNEKRRFHKIAGHYRGQCHSCCNRARQERLQRRRETQVARRAEPQRHTMLCMCCKCEARIELVVESSADDLRAFQQLFLSTLSFVCPWCASQQ

SEQ ID NO: 111 - DNA, 6379 bp, Artificial Sequence
  D-2 (overlapping-2)
  misc_feature (1368)..(1433): encodes tPA
  misc_feature (1434)..(1925): encodes FLT3L
  misc_feature (1932)..(2321): 16E6N (1-130aa)
  misc_feature (1932)..(3083): 16E6/E7
  misc_feature (2322)..(2576): 16E7N (1-85aa)
  misc_feature (2577)..(2918): 16E6C (45-158aa)
  misc_feature (2919)..(3083): 16E7C (44-98aa)
  misc_feature (3084)..(3965): 18E6/E7
taccgatgtacgggccagatatacgcgttgacattgattattgactagttattaatagtaatcaattacggggtcattagttcatagcccatatatggagttccgcgttacataacttacggtaaatggcccgcctggctgaccgcccaacgacccccgcccattgacgtcaataatgacgtatgttcccatagtaacgccaatagggactttccattgacgtcaatgggtggagtatttacggtaaactgcccacttggcagtacatcaagtgtatcatatgccaagtacgccccctattgacgtcaatgacggtaaatggcccgcctggcattatgcccagtacatgaccttatgggactttcctacttggcagtacatctacgtattagtcatcgctattaccatggtgatgcggttttggcagtacatcaatgggcgtggatagcggtttgactcacggggatttccaagtctccaccccattgacgtcaatgggagtttgttttggcaccaaaatcaacgggactttccaaaatgtcgtaacaactccgccccattgacgcaaatgggcggtaggcgtgtacggtgggaggtctatataagcagagctctctggctaactagagaacccactgcttactggcttatcgaaattaatacgactcactatagggagacccaagctggctagcgtgagtttggggacccttgattgttctttctttttcgctattgtaaaattcatgttatatggagggggcaaagttttcagggtgttgtttagaacgggaagatgtcccttgtatcaccatggaccctcatgataattttgtttctttcactttctactctgttgacaaccattgtctcctcttattttcttttcattttctgtaactttttcgttaaactttagcttgcatttgtaacgaatttttaaattcacttttgtttatttgtcagattgtaagtactttctctaatcacttttttttcaaggcaatcagggtatattatattgtacttcagcacagttttagagaacaattgttataattaaatgataaggtagaatatttctgcatataaattctggctggcgtggaaatattcttattggtagaaacaactacatcctggtcatcatcctgcctttctctttatggttacaatgatatacactgtttgagatgaggataaaatactctgagtccaaaccgggcccctctgctaaccatgttcatgccttcttctttttcctacagctcctgggcaacgtgctggttattgtgctgtctcatcattttggcaaagaattgtaatacgactcactatagggcgaattgaagcttggtaccgccaccatggatgctatgaaacggggcctgtgctgcgtgctgctcctgtgcggcgctgtgtttgtgagccctagcatcacccaggactgctccttccaacacagccccatctcctccgacttcgctgtcaaaatccgtgagctgtctgactacctgcttcaagattacccagtcaccgtggcctccaacctgcaggacgaggagctctgcgggggcctctggcggctggtcctggcacagcgctggatggagcggctcaagactgtcgctgggtccaagatgcaaggcttgctggagcgcgtgaacacggagatacactttgtcaccaaatgtgcctttcagcccccccccagctgtcttcgcttcgtccagaccaacatctcccgcctcctgcaggagacctccgagcagctggtggcgctgaagccctggatcactcgccagaacttctcccggtgcctggagctgcagtgtcagcccgactcctcaaccctgccacccccatggagtccccggcccctggaggccacagccccgacagccccgggcggcggcagcggcgatgctagcatgcaccagaagagaaccgccatgttccaggaccctcaggagagacctaggaagctgcctcacctgtgtacagagctccagacaaccatccacgacatcatcctggagtgcgtgtactgtaagcagcagctgctgagaagagaggtgtacgacttcgccttcagagacctgtgcatcgtgtacagagacggcaacccttacgccgtgtgcgataagtgtctgaagttctattccaagatctctgagtacagatactactgctactctgtgtacggcaccacactggagcagcagtacaacaagcctctgtgcgacctcctgatccgctgcatcaactgccagaagcctctgtgccctgaggagaagcagagacacctggacaagaagcagatgcacggcgacacccctaccctgcacgagtacatgctggacctccagcctgagaccacagacctgtactgctacgagcagctgaacgacagctctgaggaagaggacgagattgacggacctgctggccaggccgagcctgacagagcccactacaatatcgtgacattctgttgcaagtgcgactctaccctgagactgtgcgtgcagtctacccacgtggacatcagaaccctggaggacctgctgatgggcctgagaagagaggtgtacgacttcgccttcagagacctgtgcatcgtgtacagagacggcaacccttacgccgtgtgcgataagtgtctgaagttctattccaagatctctgagtacagatactactgctactctgtgtacggcaccacactggagcagcagtacaacaagcctctgtgcgacctcctgatccgctgcatcaactgccagaagcctctgtgccctgaggagaagcagagacacctggacaagaagcagcggttccacaacatcagaggcagatggaccggcaggtgcatgtcctgctgtagatcctccagaaccagacgggagacccagctgcaggccgagcctgacagagcccactacaatatcgtgacattctgttgcaagtgcgactctaccctgagactgtgcgtgcagtctacccacgtggacatcagaaccctggaggacctgctgatgggcaccctgggcatcgtgtgccctatctgctctcagaagcctatggccaggttcgaggaccctaccagaagaccctacaagctgcctgacctgtgcaccgagctgaacacctctctgcaagacatcgagatcacctgcgtgtactgcaagaccgtgctggagctgaccgaggtgttcgagttcgccttcaaggacctgttcgtggtgtacagagacagcatccctcacgctgcctgccacaagtgcatcgacttctattccaggatcagggagctgcgctattactccgactctgtgatgtacggccccaaggccaccctccaggacatcgtgctgcacctggagcctcagaacgagatccccgtggacctgctgtgccacgagcagctgtctgactctgaagaggagaacgacgagatcgacggcgtgaaccaccagcacctgcctgccaggagagctgaaccccagcggcataccatgctgtgtatgtgcttctactctaggatcagagagctgaggtactactctgactctgtgtacggcgacaccctggagaagctgaccaacaccggcctgtacaacctgctgatccggtgcctgaggtgccagaagcctctgaaccctgccgagaagctgagacacctgaacgagaagagaagattccacaagatcgctggccactacagaggccagtgccactcttgctgcaacagagccagacaggagagactccagcggagaagggagacccaggtggccagaagagccgagcctcagagacacaccatgctgtgcatgtgctgcaagtgcgaggccagaatcgagctggtggtggagagctctgccgacgacctgagagccttccagcagctgttcctgtctaccctgagcttcgtgtgcccttggtgcgcctctcagcagtaatctagagtcggggcggccggccgcttcgagcagacatgataagatacattgatgagtttggacaaaccacaactagaatgcagtgaaaaaaatgctttatttgtgaaatttgtgatgctattgctttatttgtaaccattataagctgcaataaacaagttaacaacaacaattgcattcattttatgtttcaggttcagggggaggtgtgggaggttttttaaagcaagtaaaacctctacaaatgtggtaaaatcgataaggatctgaacgatggagcggagaatgggcggaactgggcggagttaggggcgggatgggcggagttaggggcgggactatggttgctgactaattgagatgcatgctttgcatacttctgcctgctggggagcctggggactttccacacctggttgctgactaattgagatgcatgctttgcatacttctgcctgctggggagcctggggactttccacaccctaactgacacacattccacagcggatccgtcgacttcagaagaactcgtcaagaaggcgatagaaggcgatgcgccgcgaatcgggagcggcgataccgtagagcacgaggaagcggtcagcccattcgccgccaagctcttcagcaatatcacgggtagccaacgctatgtcctgatagcggtccgccacacccagccggccacagtcgatgaatccagaaaagcggccattttccaccatgatattcggcaagcaggcatcgccatgggtcacgacgagatcctcgccgtcgggcatgctcgccttgagcctggcgaacagttcggctggcgcgagcccctgatgctcttcgtccagatcatcctgatcgacaagaccggcttccatccgagtacgtgctcgctcgatgcgatgtttcgcttggtggtcgaatgggcaggtagccggatcaagcgtatgcagccgccgcattgcatcagccatgatggatactttctcggcaggagcaaggtgagatgacaggagatcctgccccggcacttcgcccaatagcagccagtcccttcccgcttcagtgacaacgtcgagcacagctgcgcaaggaacgcccgtcgtggccagccacgatagccgcgctgcctcgtcttgcagttcattcagggcaccggacaggtcggtcttgacaaaaagaaccgggcgcccctgcgctgacagccggaacacggcggcatcagagcagccgattgtctgttgtgcccagtcatagccgaatagcctctccacccaagcggccggagaacctgcgtgcaatccatcttgttcaatcatgcgaaacgatcctcatcctgtctcttgatcagatcttgatcccctgcgccatcagatccttggcggcaagaaagccatccagtttactttgcagggcttcccaaccttaccagagggcgccccagctggcaattccggttcgcttgctgtccataaaaccgcccagtctagctatcgccatgtaagcccactgcaagctacctgctttctctttgcgcttgcgttttcccttgtccagatagcccagtagctgacattcatccggggtcagcaccgtttctgcggactggctttctacgtgaaaaggatctaggtgaagatcctttttgataatctcatgaccaaaatcccttaacgtgagttttcgttccactgagcgtcagaccccgtagaaaagatcaaaggatcttcttgagatcctttttttctgcgcgtaatctgctgcttgcaaacaaaaaaaccaccgctaccagcggtggtttgtttgccggatcaagagctaccaactctttttccgaaggtaactggcttcagcagagcgcagataccaaatactgttcttctagtgtagccgtagttaggccaccacttcaagaactctgtagcaccgcctacatacctcgctctgctaatcctgttaccagtggctgctgccagtggcgataagtcgtgtcttaccgggttggactcaagacgatagttaccggataaggcgcagcggtcgggctgaacggggggttcgtgcacacagcccagcttggagcgaacgacctacaccgaactgagatacctacagcgtgagctatgagaaagcgccacgcttcccgaagggagaaaggcggacaggtatccggtaagcggcagggtcggaacaggagagcgcacgagggagcttccagggggaaacgcccggtatctttatagtcctgtcgggtttcgccacctctgacttgagcgtcgatttttgtgatgctcgtcaggggggcggagcctatggaaaaacgccagcaacgcggcctttttacggttcctggccttttgctggccttttgctcacatgttcgggcccaatcgacccgggcgacggccagtgaattg

SEQ ID NO: 112 - protein, 865 aa, Artificial Sequence
  D-2
MDAMKRGLCCVLLLCGAVFVSPSITQDCSFQHSPISSDFAVKIRELSDYLLQDYPVTVASNLQDEELCGGLWRLVLAQRWMERLKTVAGSKMQGLLERVNTEIHFVTKCAFQPPPSCLRFVQTNISRLLQETSEQLVALKPWITRQNFSRCLELQCQPDSSTLPPPWSPRPLEATAPTAPGGGSGDASMHQKRTAMFQDPQERPRKLPHLCTELQTTIHDIILECVYCKQQLLRREVYDFAFRDLCIVYRDGNPYAVCDKCLKFYSKISEYRYYCYSVYGTTLEQQYNKPLCDLLIRCINCQKPLCPEEKQRHLDKKQMHGDTPTLHEYMLDLQPETTDLYCYEQLNDSSEEEDEIDGPAGQAEPDRAHYNIVTFCCKCDSTLRLCVQSTHVDIRTLEDLLMGLRREVYDFAFRDLCIVYRDGNPYAVCDKCLKFYSKISEYRYYCYSVYGTTLEQQYNKPLCDLLIRCINCQKPLCPEEKQRHLDKKQRFHNIRGRWTGRCMSCCRSSRTRRETQLQAEPDRAHYNIVTFCCKCDSTLRLCVQSTHVDIRTLEDLLMGTLGIVCPICSQKPMARFEDPTRRPYKLPDLCTELNTSLQDIEITCVYCKTVLELTEVFEFAFKDLFVVYRDSIPHAACHKCIDFYSRIRELRYYSDSVMYGPKATLQDIVLHLEPQNEIPVDLLCHEQLSDSEEENDEIDGVNHQHLPARRAEPQRHTMLCMCFYSRIRELRYYSDSVYGDTLEKLTNTGLYNLLIRCLRCQKPLNPAEKLRHLNEKRRFHKIAGHYRGQCHSCCNRARQERLQRRRETQVARRAEPQRHTMLCMCCKCEARIELVVESSADDLRAFQQLFLSTLSFVCPWCASQQ

SEQ ID NO: 113 - DNA, 6085 bp, Artificial Sequence
  E-1 (Order-1)
  misc_feature (1368)..(1433): encodes tPA
  misc_feature (1434)..(1925): encodes FLT3L
  misc_feature (1932)..(2186): 16E6N
  misc_feature (1932)..(2789): 16E6/E7
  misc_feature (2187)..(2330): 16E7C
  misc_feature (2331)..(2525): 16E7N
  misc_feature (2526)..(2789): 16E6C
  misc_feature (2790)..(3671): 18E6/E7
taccgatgtacgggccagatatacgcgttgacattgattattgactagttattaatagtaatcaattacggggtcattagttcatagcccatatatggagttccgcgttacataacttacggtaaatggcccgcctggctgaccgcccaacgacccccgcccattgacgtcaataatgacgtatgttcccatagtaacgccaatagggactttccattgacgtcaatgggtggagtatttacggtaaactgcccacttggcagtacatcaagtgtatcatatgccaagtacgccccctattgacgtcaatgacggtaaatggcccgcctggcattatgcccagtacatgaccttatgggactttcctacttggcagtacatctacgtattagtcatcgctattaccatggtgatgcggttttggcagtacatcaatgggcgtggatagcggtttgactcacggggatttccaagtctccaccccattgacgtcaatgggagtttgttttggcaccaaaatcaacgggactttccaaaatgtcgtaacaactccgccccattgacgcaaatgggcggtaggcgtgtacggtgggaggtctatataagcagagctctctggctaactagagaacccactgcttactggcttatcgaaattaatacgactcactatagggagacccaagctggctagcgtgagtttggggacccttgattgttctttctttttcgctattgtaaaattcatgttatatggagggggcaaagttttcagggtgttgtttagaacgggaagatgtcccttgtatcaccatggaccctcatgataattttgtttctttcactttctactctgttgacaaccattgtctcctcttattttcttttcattttctgtaactttttcgttaaactttagcttgcatttgtaacgaatttttaaattcacttttgtttatttgtcagattgtaagtactttctctaatcacttttttttcaaggcaatcagggtatattatattgtacttcagcacagttttagagaacaattgttataattaaatgataaggtagaatatttctgcatataaattctggctggcgtggaaatattcttattggtagaaacaactacatcctggtcatcatcctgcctttctctttatggttacaatgatatacactgtttgagatgaggataaaatactctgagtccaaaccgggcccctctgctaaccatgttcatgccttcttctttttcctacagctcctgggcaacgtgctggttattgtgctgtctcatcattttggcaaagaattgtaatacgactcactatagggcgaattgaagcttggtaccgccaccatggatgctatgaaacggggcctgtgctgcgtgctgctcctgtgcggcgctgtgtttgtgagccctagcatcacccaggactgctccttccaacacagccccatctcctccgacttcgctgtcaaaatccgtgagctgtctgactacctgcttcaagattacccagtcaccgtggcctccaacctgcaggacgaggagctctgcgggggcctctggcggctggtcctggcacagcgctggatggagcggctcaagactgtcgctgggtccaagatgcaaggcttgctggagcgcgtgaacacggagatacactttgtcaccaaatgtgcctttcagcccccccccagctgtcttcgcttcgtccagaccaacatctcccgcctcctgcaggagacctccgagcagctggtggcgctgaagccctggatcactcgccagaacttctcccggtgcctggagctgcagtgtcagcccgactcctcaaccctgccacccccatggagtccccggcccctggaggccacagccccgacagccccgggcggcggcagcggcgatgctagcatgcaccagaagagaaccgccatgttccaggaccctcaggagagacctaggaagctgcctcacctgtgtacagagctccagacaaccatccacgacatcatcctggagtgcgtgtactgtaagcagcagctgctgagaagagaggtgtacgacttcgccttcagagacctgtgcatcgtgtacagagacggcaacccttacgccgtgtgcgataagtgtctgaagttctattccaaaatctccgaatataggtaccactacaacatcgtgaccttctgctgcaagtgcgactctaccctgagactgtgcgtgcagtctacccacgtggacatcagaaccctggaggacctgctgatgggcaccctgggcatcgtgtgccctatctgctctcagaagcctatgcacggcgacacccctaccctgcacgagtacatgctggacctccagcctgagaccacagacctgtactgctacgagcagctgaacgacagctctgaggaagaggacgagattgacggacctgctggccaggccgagcctgacagagcccactacaatatcgtgacattctgttgcaaatgcgactccacactggacaagtgcctgaagttctacagcaagatctctgagtacagatactactgctactctgtgtacggcaccacactggagcagcagtacaacaagcctctgtgcgacctcctgatccgctgcatcaactgccagaagcctctgtgccctgaggagaagcagagacacctggacaagaagcagcggttccacaacatcagaggcagatggaccggcaggtgcatgtcctgctgtagatcctccagaaccagacgggagacccagctgatggccaggttcgaggaccctaccagaagaccctacaagctgcctgacctgtgcaccgagctgaacacctctctgcaagacatcgagatcacctgcgtgtactgcaagaccgtgctggagctgaccgaggtgttcgagttcgccttcaaggacctgttcgtggtgtacagagacagcatccctcacgctgcctgccacaagtgcatcgacttctattccaggatcagggagctgcgctattactccgactctgtgatgtacggccccaaggccaccctccaggacatcgtgctgcacctggagcctcagaacgagatccccgtggacctgctgtgccacgagcagctgtctgactctgaagaggagaacgacgagatcgacggcgtgaaccaccagcacctgcctgccaggagagctgaaccccagcggcataccatgctgtgtatgtgcttctactctaggatcagagagctgaggtactactctgactctgtgtacggcgacaccctggagaagctgaccaacaccggcctgtacaacctgctgatccggtgcctgaggtgccagaagcctctgaaccctgccgagaagctgagacacctgaacgagaagagaagattccacaagatcgctggccactacagaggccagtgccactcttgctgcaacagagccagacaggagagactccagcggagaagggagacccaggtggccagaagagccgagcctcagagacacaccatgctgtgcatgtgctgcaagtgcgaggccagaatcgagctggtggtggagagctctgccgacgacctgagagccttccagcagctgttcctgtctaccctgagcttcgtgtgcccttggtgcgcctctcagcagtaatctagagtcggggcggccggccgcttcgagcagacatgataagatacattgatgagtttggacaaaccacaactagaatgcagtgaaaaaaatgctttatttgtgaaatttgtgatgctattgctttatttgtaaccattataagctgcaataaacaagttaacaacaacaattgcattcattttatgtttcaggttcagggggaggtgtgggaggttttttaaagcaagtaaaacctctacaaatgtggtaaaatcgataaggatctgaacgatggagcggagaatgggcggaactgggcggagttaggggcgggatgggcggagttaggggcgggactatggttgctgactaattgagatgcatgctttgcatacttctgcctgctggggagcctggggactttccacacctggttgctgactaattgagatgcatgctttgcatacttctgcctgctggggagcctggggactttccacaccctaactgacacacattccacagcggatccgtcgacttcagaagaactcgtcaagaaggcgatagaaggcgatgcgccgcgaatcgggagcggcgataccgtagagcacgaggaagcggtcagcccattcgccgccaagctcttcagcaatatcacgggtagccaacgctatgtcctgatagcggtccgccacacccagccggccacagtcgatgaatccagaaaagcggccattttccaccatgatattcggcaagcaggcatcgccatgggtcacgacgagatcctcgccgtcgggcatgctcgccttgagcctggcgaacagttcggctggcgcgagcccctgatgctcttcgtccagatcatcctgatcgacaagaccggcttccatccgagtacgtgctcgctcgatgcgatgtttcgcttggtggtcgaatgggcaggtagccggatcaagcgtatgcagccgccgcattgcatcagccatgatggatactttctcggcaggagcaaggtgagatgacaggagatcctgccccggcacttcgcccaatagcagccagtcccttcccgcttcagtgacaacgtcgagcacagctgcgcaaggaacgcccgtcgtggccagccacgatagccgcgctgcctcgtcttgcagttcattcagggcaccggacaggtcggtcttgacaaaaagaaccgggcgcccctgcgctgacagccggaacacggcggcatcagagcagccgattgtctgttgtgcccagtcatagccgaatagcctctccacccaagcggccggagaacctgcgtgcaatccatcttgttcaatcatgcgaaacgatcctcatcctgtctcttgatcagatcttgatcccctgcgccatcagatccttggcggcaagaaagccatccagtttactttgcagggcttcccaaccttaccagagggcgccccagctggcaattccggttcgcttgctgtccataaaaccgcccagtctagctatcgccatgtaagcccactgcaagctacctgctttctctttgcgcttgcgttttcccttgtccagatagcccagtagctgacattcatccggggtcagcaccgtttctgcggactggctttctacgtgaaaaggatctaggtgaagatcctttttgataatctcatgaccaaaatcccttaacgtgagttttcgttccactgagcgtcagaccccgtagaaaagatcaaaggatcttcttgagatcctttttttctgcgcgtaatctgctgcttgcaaacaaaaaaaccaccgctaccagcggtggtttgtttgccggatcaagagctaccaactctttttccgaaggtaactggcttcagcagagcgcagataccaaatactgttcttctagtgtagccgtagttaggccaccacttcaagaactctgtagcaccgcctacatacctcgctctgctaatcctgttaccagtggctgctgccagtggcgataagtcgtgtcttaccgggttggactcaagacgatagttaccggataaggcgcagcggtcgggctgaacggggggttcgtgcacacagcccagcttggagcgaacgacctacaccgaactgagatacctacagcgtgagctatgagaaagcgccacgcttcccgaagggagaaaggcggacaggtatccggtaagcggcagggtcggaacaggagagcgcacgagggagcttccagggggaaacgcccggtatctttatagtcctgtcgggtttcgccacctctgacttgagcgtcgatttttgtgatgctcgtcaggggggcggagcctatggaaaaacgccagcaacgcggcctttttacggttcctggccttttgctggccttttgctcacatgttcgggcccaatcgacccgggcgacggccagtgaattg

SEQ ID NO: 114 - protein, 767 aa, Artificial Sequence
  E-1
MDAMKRGLCCVLLLCGAVFVSPSITQDCSFQHSPISSDFAVKIRELSDYLLQDYPVTVASNLQDEELCGGLWRLVLAQRWMERLKTVAGSKMQGLLERVNTEIHFVTKCAFQPPPSCLRFVQTNISRLLQETSEQLVALKPWITRQNFSRCLELQCQPDSSTLPPPWSPRPLEATAPTAPGGGSGDASMHQKRTAMFQDPQERPRKLPHLCTELQTTIHDIILECVYCKQQLLRREVYDFAFRDLCIVYRDGNPYAVCDKCLKFYSKISEYRYHYNIVTFCCKCDSTLRLCVQSTHVDIRTLEDLLMGTLGIVCPICSQKPMHGDTPTLHEYMLDLQPETTDLYCYEQLNDSSEEEDEIDGPAGQAEPDRAHYNIVTFCCKCDSTLDKCLKFYSKISEYRYYCYSVYGTTLEQQYNKPLCDLLIRCINCQKPLCPEEKQRHLDKKQRFHNIRGRWTGRCMSCCRSSRTRRETQLMARFEDPTRRPYKLPDLCTELNTSLQDIEITCVYCKTVLELTEVFEFAFKDLFVVYRDSIPHAACHKCIDFYSRIRELRYYSDSVMYGPKATLQDIVLHLEPQNEIPVDLLCHEQLSDSEEENDEIDGVNHQHLPARRAEPQRHTMLCMCFYSRIRELRYYSDSVYGDTLEKLTNTGLYNLLIRCLRCQKPLNPAEKLRHLNEKRRFHKIAGHYRGQCHSCCNRARQERLQRRRETQVARRAEPQRHTMLCMCCKCEARIELVVESSADDLRAFQQLFLSTLSFVCPWCASQQ

SEQ ID NO: 115 - DNA, 6085 bp, Artificial Sequence
  E-2 (Order-2)
  misc_feature (1368)..(1433): encodes tPA
  misc_feature (1434)..(1925): encodes FLT3L
  misc_feature (1932)..(2195): 16E6C
  misc_feature (1932)..(2789): 16E6/E7
  misc_feature (2196)..(2339): 16E7C
  misc_feature (2340)..(2594): 16E6N
  misc_feature (2595)..(2789): 16E7N
  misc_feature (2790)..(3671): 18E6/E7
taccgatgtacgggccagatatacgcgttgacattgattattgactagttattaatagtaatcaattacggggtcattagttcatagcccatatatggagttccgcgttacataacttacggtaaatggcccgcctggctgaccgcccaacgacccccgcccattgacgtcaataatgacgtatgttcccatagtaacgccaatagggactttccattgacgtcaatgggtggagtatttacggtaaactgcccacttggcagtacatcaagtgtatcatatgccaagtacgccccctattgacgtcaatgacggtaaatggcccgcctggcattatgcccagtacatgaccttatgggactttcctacttggcagtacatctacgtattagtcatcgctattaccatggtgatgcggttttggcagtacatcaatgggcgtggatagcggtttgactcacggggatttccaagtctccaccccattgacgtcaatgggagtttgttttggcaccaaaatcaacgggactttccaaaatgtcgtaacaactccgccccattgacgcaaatgggcggtaggcgtgtacggtgggaggtctatataagcagagctctctggctaactagagaacccactgcttactggcttatcgaaattaatacgactcactatagggagacccaagctggctagcgtgagtttggggacccttgattgttctttctttttcgctattgtaaaattcatgttatatggagggggcaaagttttcagggtgttgtttagaacgggaagatgtcccttgtatcaccatggaccctcatgataattttgtttctttcactttctactctgttgacaaccattgtctcctcttattttcttttcattttctgtaactttttcgttaaactttagcttgcatttgtaacgaatttttaaattcacttttgtttatttgtcagattgtaagtactttctctaatcacttttttttcaaggcaatcagggtatattatattgtacttcagcacagttttagagaacaattgttataattaaatgataaggtagaatatttctgcatataaattctggctggcgtggaaatattcttattggtagaaacaactacatcctggtcatcatcctgcctttctctttatggttacaatgatatacactgtttgagatgaggataaaatactctgagtccaaaccgggcccctctgctaaccatgttcatgccttcttctttttcctacagctcctgggcaacgtgctggttattgtgctgtctcatcattttggcaaagaattgtaatacgactcactatagggcgaattgaagcttggtaccgccaccatggatgctatgaaacggggcctgtgctgcgtgctgctcctgtgcggcgctgtgtttgtgagccctagcatcacccaggactgctccttccaacacagccccatctcctccgacttcgctgtcaaaatccgtgagctgtctgactacctgcttcaagattacccagtcaccgtggcctccaacctgcaggacgaggagctctgcgggggcctctggcggctggtcctggcacagcgctggatggagcggctcaagactgtcgctgggtccaagatgcaaggcttgctggagcgcgtgaacacggagatacactttgtcaccaaatgtgcctttcagcccccccccagctgtcttcgcttcgtccagaccaacatctcccgcctcctgcaggagacctccgagcagctggtggcgctgaagccctggatcactcgccagaacttctcccggtgcctggagctgcagtgtcagcccgactcctcaaccctgccacccccatggagtccccggcccctggaggccacagccccgacagccccgggcggcggcagcggcgatgctagcgacaagtgcctgaagttctacagcaagatctctgagtacagatactactgctactctgtgtacggcaccacactggagcagcagtacaacaagcctctgtgcgacctcctgatccgctgcatcaactgccagaagcctctgtgccctgaggagaagcagagacacctggacaagaagcagcggttccacaacatcagaggcagatggaccggcaggtgcatgtcctgctgtagatcctccagaaccagacgggagacccagctgcactacaacatcgtgaccttctgctgcaagtgcgactctaccctgagactgtgcgtgcagtctacccacgtggacatcagaaccctggaggacctgctgatgggcaccctgggcatcgtgtgccctatctgctctcagaagcctatgcaccagaagagaaccgccatgttccaggaccctcaggagagacctaggaagctgcctcacctgtgtacagagctccagacaaccatccacgacatcatcctggagtgcgtgtactgtaagcagcagctgctgagaagagaggtgtacgacttcgccttcagagacctgtgcatcgtgtacagagacggcaacccttacgccgtgtgcgataagtgtctgaagttctattccaaaatctccgaatataggtacatgcacggcgacacccctaccctgcacgagtacatgctggacctccagcctgagaccacagacctgtactgctacgagcagctgaacgacagctctgaggaagaggacgagattgacggacctgctggccaggccgagcctgacagagcccactacaatatcgtgacattctgttgcaaatgcgactccacactgatggccaggttcgaggaccctaccagaagaccctacaagctgcctgacctgtgcaccgagctgaacacctctctgcaagacatcgagatcacctgcgtgtactgcaagaccgtgctggagctgaccgaggtgttcgagttcgccttcaaggacctgttcgtggtgtacagagacagcatccctcacgctgcctgccacaagtgcatcgacttctattccaggatcagggagctgcgctattactccgactctgtgatgtacggccccaaggccaccctccaggacatcgtgctgcacctggagcctcagaacgagatccccgtggacctgctgtgccacgagcagctgtctgactctgaagaggagaacgacgagatcgacggcgtgaaccaccagcacctgcctgccaggagagctgaaccccagcggcataccatgctgtgtatgtgcttctactctaggatcagagagctgaggtactactctgactctgtgtacggcgacaccctggagaagctgaccaacaccggcctgtacaacctgctgatccggtgcctgaggtgccagaagcctctgaaccctgccgagaagctgagacacctgaacgagaagagaagattccacaagatcgctggccactacagaggccagtgccactcttgctgcaacagagccagacaggagagactccagcggagaagggagacccaggtggccagaagagccgagcctcagagacacaccatgctgtgcatgtgctgcaagtgcgaggccagaatcgagctggtggtggagagctctgccgacgacctgagagccttccagcagctgttcctgtctaccctgagcttcgtgtgcccttggtgcgcctctcagcagtaatctagagtcggggcggccggccgcttcgagcagacatgataagatacattgatgagtttggacaaaccacaactagaatgcagtgaaaaaaatgctttatttgtgaaatttgtgatgctattgctttatttgtaaccattataagctgcaataaacaagttaacaacaacaattgcattcattttatgtttcaggttcagggggaggtgtgggaggttttttaaagcaagtaaaacctctacaaatgtggtaaaatcgataaggatctgaacgatggagcggagaatgggcggaactgggcggagttaggggcgggatgggcggagttaggggcgggactatggttgctgactaattgagatgcatgctttgcatacttctgcctgctggggagcctggggactttccacacctggttgctgactaattgagatgcatgctttgcatacttctgcctgctggggagcctggggactttccacaccctaactgacacacattccacagcggatccgtcgacttcagaagaactcgtcaagaaggcgatagaaggcgatgcgccgcgaatcgggagcggcgataccgtagagcacgaggaagcggtcagcccattcgccgccaagctcttcagcaatatcacgggtagccaacgctatgtcctgatagcggtccgccacacccagccggccacagtcgatgaatccagaaaagcggccattttccaccatgatattcggcaagcaggcatcgccatgggtcacgacgagatcctcgccgtcgggcatgctcgccttgagcctggcgaacagttcggctggcgcgagcccctgatgctcttcgtccagatcatcctgatcgacaagaccggcttccatccgagtacgtgctcgctcgatgcgatgtttcgcttggtggtcgaatgggcaggtagccggatcaagcgtatgcagccgccgcattgcatcagccatgatggatactttctcggcaggagcaaggtgagatgacaggagatcctgccccggcacttcgcccaatagcagccagtcccttcccgcttcagtgacaacgtcgagcacagctgcgcaaggaacgcccgtcgtggccagccacgatagccgcgctgcctcgtcttgcagttcattcagggcaccggacaggtcggtcttgacaaaaagaaccgggcgcccctgcgctgacagccggaacacggcggcatcagagcagccgattgtctgttgtgcccagtcatagccgaatagcctctccacccaagcggccggagaacctgcgtgcaatccatcttgttcaatcatgcgaaacgatcctcatcctgtctcttgatcagatcttgatcccctgcgccatcagatccttggcggcaagaaagccatccagtttactttgcagggcttcccaaccttaccagagggcgccccagctggcaattccggttcgcttgctgtccataaaaccgcccagtctagctatcgccatgtaagcccactgcaagctacctgctttctctttgcgcttgcgttttcccttgtccagatagcccagtagctgacattcatccggggtcagcaccgtttctgcggactggctttctacgtgaaaaggatctaggtgaagatcctttttgataatctcatgaccaaaatcccttaacgtgagttttcgttccactgagcgtcagaccccgtagaaaagatcaaaggatcttcttgagatcctttttttctgcgcgtaatctgctgcttgcaaacaaaaaaaccaccgctaccagcggtggtttgtttgccggatcaagagctaccaactctttttccgaaggtaactggcttcagcagagcgcagataccaaatactgttcttctagtgtagccgtagttaggccaccacttcaagaactctgtagcaccgcctacatacctcgctctgctaatcctgttaccagtggctgctgccagtggcgataagtcgtgtcttaccgggttggactcaagacgatagttaccggataaggcgcagcggtcgggctgaacggggggttcgtgcacacagcccagcttggagcgaacgacctacaccgaactgagatacctacagcgtgagctatgagaaagcgccacgcttcccgaagggagaaaggcggacaggtatccggtaagcggcagggtcggaacaggagagcgcacgagggagcttccagggggaaacgcccggtatctttatagtcctgtcgggtttcgccacctctgacttgagcgtcgatttttgtgatgctcgtcaggggggcggagcctatggaaaaacgccagcaacgcggcctttttacggttcctggccttttgctggccttttgctcacatgttcgggcccaatcgacccgggcgacggccagtgaattg

SEQ ID NO: 116 - protein, 767 aa, Artificial Sequence
  E-2
MDAMKRGLCCVLLLCGAVFVSPSITQDCSFQHSPISSDFAVKIRELSDYLLQDYPVTVASNLQDEELCGGLWRLVLAQRWMERLKTVAGSKMQGLLERVNTEIHFVTKCAFQPPPSCLRFVQTNISRLLQETSEQLVALKPWITRQNFSRCLELQCQPDSSTLPPPWSPRPLEATAPTAPGGGSGDASDKCLKFYSKISEYRYYCYSVYGTTLEQQYNKPLCDLLIRCINCQKPLCPEEKQRHLDKKQRFHNIRGRWTGRCMSCCRSSRTRRETQLHYNIVTFCCKCDSTLRLCVQSTHVDIRTLEDLLMGTLGIVCPICSQKPMHQKRTAMFQDPQERPRKLPHLCTELQTTIHDIILECVYCKQQLLRREVYDFAFRDLCIVYRDGNPYAVCDKCLKFYSKISEYRYMHGDTPTLHEYMLDLQPETTDLYCYEQLNDSSEEEDEIDGPAGQAEPDRAHYNIVTFCCKCDSTLMARFEDPTRRPYKLPDLCTELNTSLQDIEITCVYCKTVLELTEVFEFAFKDLFVVYRDSIPHAACHKCIDFYSRIRELRYYSDSVMYGPKATLQDIVLHLEPQNEIPVDLLCHEQLSDSEEENDEIDGVNHQHLPARRAEPQRHTMLCMCFYSRIRELRYYSDSVYGDTLEKLTNTGLYNLLIRCLRCQKPLNPAEKLRHLNEKRRFHKIAGHYRGQCHSCCNRARQERLQRRRETQVARRAEPQRHTMLCMCCKCEARIELVVESSADDLRAFQQLFLSTLSFVCPWCASQQ